European Patent Application EP 4 361 260 A1, published May 1, 2024. Title: Imine reductase mutant,co-expressed enzyme of imine reductase and glucose dehydrogenase,and use thereof. The sequence listing filed with the application follows.

SEQUENCE LISTING (173 sequences)

SEQ ID NO: 1 - protein, 292 aa, Artificial Sequence
MRHLSVIGLGAMGSALATTLLKAGHPVTVWNRSAAKAAPLQALGATLAPSVGAAIAASDITLVCVDNYAVSQLLLDEASDAVAGKLLVQLSTGSPQGARALESWSHARGARYLDGAILCFPAQIGTSDASIICSGASAAFSEAEPVLSLLAPTLDHVAEAVGAAAAQDCAVAAYFAGGLLGALHGALICEAEGLPVAKVCAQFSELSPILGGDVAHLGKTLASGDFDHPYASLKTWSAAISRLAGHATDAGIDSRFPRFAADLFEEGVAQGFGQQEVSALIKVLRARNGAAQ

SEQ ID NO: 2 - DNA, 879 bp, Artificial Sequence
atgcgccatctgagcgtgattggcctgggcgcgatgggcagcgcgctggcgaccaccctgctgaaggcaggacacccagtaacagtttggaatcgtagtgctgcaaaggctgctccactccaagctctaggtgctactttggctcctagtgttggagccgctatcgccgcgagcgatattaccctggtgtgcgtggataactatgcggtgagccagctgctgctggatgaagcgagcgatgcagtagccgggaagttgcttgtacaactttcgacgggaagtcctcaaggtgcacgtgcccttgagagctggagccatgcgcgcggcgcgcgctatctggatggcgcgattctgtgctttccggcgcagattggcaccagcgatgcgagcattatttgcagcggcgcgagcgcggcgtttagcgaagcggaaccggtgctgtctctcctcgctcccacactagaccacgttgccgaggctgtgggagcggccgcggctcaagactgcgcggtggcggcgtatttcgctggaggcctgctgggcgcgctgcatggcgcgctgatttgcgaagcggaaggcctgccggtggcgaaagtgtgcgcgcagtttagcgaactgagcccgattctgggcggcgatgtggcgcatctgggcaagacattggcgagcggcgatttcgaccacccgtatgcgagcctgaagacttggagcgcggcgattagccgcctggcgggccatgcgaccgatgcgggcattgatagccgctttccgcgctttgcggcggatctgtttgaagaaggcgtggcgcagggctttggccagcaggaagtgagcgcgctgattaaagtgctgcgcgcgcgcaacggcgcggcgcagtaa

SEQ ID NO: 3 - protein, 292 aa, Artificial Sequence
MRHLSVIGLGAMGSALATTLLKAGHPVTVWNRSAAKAAPLQALGATLAPSVGAAIAASDITLVCVDNYAVSQLLLDEASDAVAGKLLVQLSTGSPQGARALESWSHARGARYLDGAILCFPAQIGTSDASIICSGASAAFSEAEPVLSLLAPTLDHVAEAVGAAAAQDCAVAAYFAGGLLGALHGALICEAEGLPVAKVCAQFSELSPILGGDVAHLGKTLASGDFDHPAASLKTWSAAISRLAGHATDAGIDSRFPRFAADLFEEGVAQGFGQQEVSALIKVLRARNGAAQ

SEQ ID NO: 4 - DNA, 879 bp, Artificial Sequence
atgcgccatctgagcgtgattggcctgggcgcgatgggcagcgcgctggcgaccaccctgctgaaggcaggacacccagtaacagtttggaatcgtagtgctgcaaaggctgctccactccaagctctaggtgctactttggctcctagtgttggagccgctatcgccgcgagcgatattaccctggtgtgcgtggataactatgcggtgagccagctgctgctggatgaagcgagcgatgcagtagccgggaagttgcttgtacaactttcgacgggaagtcctcaaggtgcacgtgcccttgagagctggagccatgcgcgcggcgcgcgctatctggatggcgcgattctgtgctttccggcgcagattggcaccagcgatgcgagcattatttgcagcggcgcgagcgcggcgtttagcgaagcggaaccggtgctgtctctcctcgctcccacactagaccacgttgccgaggctgtgggagcggccgcggctcaagactgcgcggtggcggcgtatttcgctggaggcctgctgggcgcgctgcatggcgcgctgatttgcgaagcggaaggcctgccggtggcgaaagtgtgcgcgcagtttagcgaactgagcccgattctgggcggcgatgtggcgcatctgggcaagacattggcgagcggcgatttcgaccacccggcggcgagcctgaagacttggagcgcggcgattagccgcctggcgggccatgcgaccgatgcgggcattgatagccgctttccgcgctttgcggcggatctgtttgaagaaggcgtggcgcagggctttggccagcaggaagtgagcgcgctgattaaagtgctgcgcgcgcgcaacggcgcggcgcagtaa

SEQ ID NO: 5 - protein, 292 aa, Artificial Sequence
MRHLSVIGLGAMGSALATTLLKAGHPVTVWNRSAAKAAPLQALGATLAPSVGAAIAASDITLVCVDNYAVSQLLLDEASDAVAGKLLVQLSTGSPQGARALESWSHARGARYLDGAILCFPAQIGTSDASIICSGASAAFSEAEPVLSLLAPTLDHVAEAVGAAAAQDCAYAAYFAGGLLGALHGALICEAEGLPVAKVCAQFSELSPILGGDVAHLGKTLASGDFDHPYASLKTWSAAISRLAGHATDAGIDSRFPRFAADLFEEGVAQGFGQQEVSALIKVLRARNGAAQ

SEQ ID NO: 6 - DNA, 879 bp, Artificial Sequence
atgcgccatctgagcgtgattggcctgggcgcgatgggcagcgcgctggcgaccaccctgctgaaggcaggacacccagtaacagtttggaatcgtagtgctgcaaaggctgctccactccaagctctaggtgctactttggctcctagtgttggagccgctatcgccgcgagcgatattaccctggtgtgcgtggataactatgcggtgagccagctgctgctggatgaagcgagcgatgcagtagccgggaagttgcttgtacaactttcgacgggaagtcctcaaggtgcacgtgcccttgagagctggagccatgcgcgcggcgcgcgctatctggatggcgcgattctgtgctttccggcgcagattggcaccagcgatgcgagcattatttgcagcggcgcgagcgcggcgtttagcgaagcggaaccggtgctgtctctcctcgctcccacactagaccacgttgccgaggctgtgggagcggccgcggctcaagactgcgcgtacgcggcgtatttcgctggaggcctgctgggcgcgctgcatggcgcgctgatttgcgaagcggaaggcctgccggtggcgaaagtgtgcgcgcagtttagcgaactgagcccgattctgggcggcgatgtggcgcatctgggcaagacattggcgagcggcgatttcgaccacccgtatgcgagcctgaagacttggagcgcggcgattagccgcctggcgggccatgcgaccgatgcgggcattgatagccgctttccgcgctttgcggcggatctgtttgaagaaggcgtggcgcagggctttggccagcaggaagtgagcgcgctgattaaagtgctgcgcgcgcgcaacggcgcggcgcagtaa

SEQ ID NO: 7 - protein, 292 aa, Artificial Sequence
MRHLSVIGLGAMGSALATTLLKAGHPVTVWNRSAAKAAPLQALGATLAPSVGAAIAASDITLVCVDNYAVSQLLLDEASDAVAGKLLVQLSTGSPQGARALESWSHARGARYLDGAILCFPAQIGTSDASIICSGASAAFSEAEPVLSLLAPTLDHVAEAVGAAAAQDCAVAAYFAGGLLGALHGALICEAEGLPVAKVCAQFSELSPILGGDVAHLGKTLASGDFDHPTASLKTWSAAISRLAGHATDAGIDSRFPRFAADLFEEGVAQGFGQQEVSALIKVLRARNGAAQ

SEQ ID NO: 8 - DNA, 879 bp, Artificial Sequence
atgcgccatctgagcgtgattggcctgggcgcgatgggcagcgcgctggcgaccaccctgctgaaggcaggacacccagtaacagtttggaatcgtagtgctgcaaaggctgctccactccaagctctaggtgctactttggctcctagtgttggagccgctatcgccgcgagcgatattaccctggtgtgcgtggataactatgcggtgagccagctgctgctggatgaagcgagcgatgcagtagccgggaagttgcttgtacaactttcgacgggaagtcctcaaggtgcacgtgcccttgagagctggagccatgcgcgcggcgcgcgctatctggatggcgcgattctgtgctttccggcgcagattggcaccagcgatgcgagcattatttgcagcggcgcgagcgcggcgtttagcgaagcggaaccggtgctgtctctcctcgctcccacactagaccacgttgccgaggctgtgggagcggccgcggctcaagactgcgcggtggcggcgtatttcgctggaggcctgctgggcgcgctgcatggcgcgctgatttgcgaagcggaaggcctgccggtggcgaaagtgtgcgcgcagtttagcgaactgagcccgattctgggcggcgatgtggcgcatctgggcaagacattggcgagcggcgatttcgaccacccgacggcgagcctgaagacttggagcgcggcgattagccgcctggcgggccatgcgaccgatgcgggcattgatagccgctttccgcgctttgcggcggatctgtttgaagaaggcgtggcgcagggctttggccagcaggaagtgagcgcgctgattaaagtgctgcgcgcgcgcaacggcgcggcgcagtaa

SEQ ID NO: 9 - protein, 292 aa, Artificial Sequence
MRHLSVIGLGAMGSALATTLLKAGHPVTVWNRSAAKAAPLQALGATLAPSVGAAIAASDITLVCVDNYAVSQLLLDEASDAVAGKLLVQLSTGSPQGARALESWSHARGARYLDGAILCFPAQIGTSDASIICSGASAAFSEAEPVLSLLAPTLDHVAEAVGAAAAQDCAVAAYFAGGLLGALHGALICEAEGLPVAKVCAQFSELSPILGGDVAHLGKTLASGDFDHPGASLKTWSAAISRLAGHATDAGIDSRFPRFAADLFEEGVAQGFGQQEVSALIKVLRARNGAAQ

SEQ ID NO: 10 - DNA, 879 bp, Artificial Sequence
atgcgccatctgagcgtgattggcctgggcgcgatgggcagcgcgctggcgaccaccctgctgaaggcaggacacccagtaacagtttggaatcgtagtgctgcaaaggctgctccactccaagctctaggtgctactttggctcctagtgttggagccgctatcgccgcgagcgatattaccctggtgtgcgtggataactatgcggtgagccagctgctgctggatgaagcgagcgatgcagtagccgggaagttgcttgtacaactttcgacgggaagtcctcaaggtgcacgtgcccttgagagctggagccatgcgcgcggcgcgcgctatctggatggcgcgattctgtgctttccggcgcagattggcaccagcgatgcgagcattatttgcagcggcgcgagcgcggcgtttagcgaagcggaaccggtgctgtctctcctcgctcccacactagaccacgttgccgaggctgtgggagcggccgcggctcaagactgcgcggtggcggcgtatttcgctggaggcctgctgggcgcgctgcatggcgcgctgatttgcgaagcggaaggcctgccggtggcgaaagtgtgcgcgcagtttagcgaactgagcccgattctgggcggcgatgtggcgcatctgggcaagacattggcgagcggcgatttcgaccacccgggcgcgagcctgaagacttggagcgcggcgattagccgcctggcgggccatgcgaccgatgcgggcattgatagccgctttccgcgctttgcggcggatctgtttgaagaaggcgtggcgcagggctttggccagcaggaagtgagcgcgctgattaaagtgctgcgcgcgcgcaacggcgcggcgcagtaa

SEQ ID NO: 11 - protein, 292 aa, Artificial Sequence
MRHLSVIGLGAMGSALATTLLKAGHPVTVWNRSAAKAAPLQALGATLAPSVGAAIAASDITLVCVDNYAVSQLLLDEASDAVAGKLLVQLSTGSPQGARALESWSHARGARYLDGAILCFPAQIGTSDASIICSGASAAFSEAEPVLSLLAPTLDHVAEAVGAAAAQDCANAAYFAGGLLGALHGALICEAEGLPVAKVCAQFSELSPILGGDVAHLGKTLASGDFDHPYASLKTWSAAISRLAGHATDAGIDSRFPRFAADLFEEGVAQGFGQQEVSALIKVLRARNGAAQ

SEQ ID NO: 12 - DNA, 879 bp, Artificial Sequence
atgcgccatctgagcgtgattggcctgggcgcgatgggcagcgcgctggcgaccaccctgctgaaggcaggacacccagtaacagtttggaatcgtagtgctgcaaaggctgctccactccaagctctaggtgctactttggctcctagtgttggagccgctatcgccgcgagcgatattaccctggtgtgcgtggataactatgcggtgagccagctgctgctggatgaagcgagcgatgcagtagccgggaagttgcttgtacaactttcgacgggaagtcctcaaggtgcacgtgcccttgagagctggagccatgcgcgcggcgcgcgctatctggatggcgcgattctgtgctttccggcgcagattggcaccagcgatgcgagcattatttgcagcggcgcgagcgcggcgtttagcgaagcggaaccggtgctgtctctcctcgctcccacactagaccacgttgccgaggctgtgggagcggccgcggctcaagactgcgcgaacgcggcgtatttcgctggaggcctgctgggcgcgctgcatggcgcgctgatttgcgaagcggaaggcctgccggtggcgaaagtgtgcgcgcagtttagcgaactgagcccgattctgggcggcgatgtggcgcatctgggcaagacattggcgagcggcgatttcgaccacccgtatgcgagcctgaagacttggagcgcggcgattagccgcctggcgggccatgcgaccgatgcgggcattgatagccgctttccgcgctttgcggcggatctgtttgaagaaggcgtggcgcagggctttggccagcaggaagtgagcgcgctgattaaagtgctgcgcgcgcgcaacggcgcggcgcagtaa

SEQ ID NO: 13 - protein, 292 aa, Artificial Sequence
MRHLSVIGLGAMGSALATTLLKAGHPVTVWNRSAAKAAPLQALGATLAPSVGAAIAASDITLVCVDNYAVSQLLLDEASDAVAGKLLVQLSTGSPQGARALESWSHARGARYLDGAILCFPAQIGTSDASIICSGASAAFSEAEPVLSLLAPTLDHVAEAVGAAAAQDCAVFAYFAGGLLGALHGALICEAEGLPVAKVCAQFSELSPILGGDVAHLGKTLASGDFDHPYASLKTWSAAISRLAGHATDAGIDSRFPRFAADLFEEGVAQGFGQQEVSALIKVLRARNGAAQ

SEQ ID NO: 14 - DNA, 879 bp, Artificial Sequence
atgcgccatctgagcgtgattggcctgggcgcgatgggcagcgcgctggcgaccaccctgctgaaggcaggacacccagtaacagtttggaatcgtagtgctgcaaaggctgctccactccaagctctaggtgctactttggctcctagtgttggagccgctatcgccgcgagcgatattaccctggtgtgcgtggataactatgcggtgagccagctgctgctggatgaagcgagcgatgcagtagccgggaagttgcttgtacaactttcgacgggaagtcctcaaggtgcacgtgcccttgagagctggagccatgcgcgcggcgcgcgctatctggatggcgcgattctgtgctttccggcgcagattggcaccagcgatgcgagcattatttgcagcggcgcgagcgcggcgtttagcgaagcggaaccggtgctgtctctcctcgctcccacactagaccacgttgccgaggctgtgggagcggccgcggctcaagactgcgcggtgtttgcgtatttcgctggaggcctgctgggcgcgctgcatggcgcgctgatttgcgaagcggaaggcctgccggtggcgaaagtgtgcgcgcagtttagcgaactgagcccgattctgggcggcgatgtggcgcatctgggcaagacattggcgagcggcgatttcgaccacccgtatgcgagcctgaagacttggagcgcggcgattagccgcctggcgggccatgcgaccgatgcgggcattgatagccgctttccgcgctttgcggcggatctgtttgaagaaggcgtggcgcagggctttggccagcaggaagtgagcgcgctgattaaagtgctgcgcgcgcgcaacggcgcggcgcagtaa

SEQ ID NO: 15 - protein, 292 aa, Artificial Sequence
MRHLSVIGLGAMGSALATTLLKAGHPVTVWNRSAAKAAPLQALGATLAPSVGAAIAASDITLVCVDNYAVSQLLLDEASDAVAGKLLVQLSTGSPQGARALESWSHARGARYLDGAIVCFPAQIGTSDACIICSGASAAFSEAEPVLSLLAPTLDHVAEAVGAAAAQDCAVAAYFAGGLLGALHGALICEAEGLPVAKVCAQFSELSPFLGGDVAHLGKTLASGDFDHPYASLWTWSAAISRLAGHATDAGIDSRFPRFAADLFEEGVAQGFGQQEVSALIKVLRARNGAAQ

SEQ ID NO: 16 - DNA, 879 bp, Artificial Sequence
atgcgccatctgagcgtgattggcctgggcgcgatgggcagcgcgctggcgaccaccctgctgaaggcaggacacccagtaacagtttggaatcgtagtgctgcaaaggctgctccactccaagctctaggtgctactttggctcctagtgttggagccgctatcgccgcgagcgatattaccctggtgtgcgtggataactatgcggtgagccagctgctgctggatgaagcgagcgatgcagtagccgggaagttgcttgtacaactttcgacgggaagtcctcaaggtgcacgtgcccttgagagctggagccatgcgcgcggcgcgcgctatctggatggcgcgattgtttgctttccggcgcagattggcaccagcgatgcgtgtattatttgcagcggcgcgagcgcggcgtttagcgaagcggaaccggtgctgtctctcctcgctcccacactagaccacgttgccgaggctgtgggagcggccgcggctcaagactgcgcggtggcggcgtatttcgctggaggcctgctgggcgcgctgcatggcgcgctgatttgcgaagcggaaggcctgccggtggcgaaagtgtgcgcgcagtttagcgaactgagcccgtttctgggcggcgatgtggcgcatctgggcaagacattggcgagcggcgatttcgaccacccgtatgcgagcctgtggacttggagcgcggcgattagccgcctggcgggccatgcgaccgatgcgggcattgatagccgctttccgcgctttgcggcggatctgtttgaagaaggcgtggcgcagggctttggccagcaggaagtgagcgcgctgattaaagtgctgcgcgcgcgcaacggcgcggcgcagtaa

SEQ ID NO: 17 - protein, 292 aa, Artificial Sequence
MRHLSVIGLGAMGVALATTLLKAGHPVTVWNRSAAKAAPLQALGATLAPSVGAAIAASDITLVCVDNYAVSQLLLDEASDAVAGKLLVQLSTGSPQGARALESWSHARGARYLDGAILCFPAQIGTSDASIICSGASAAFSEAEPVLSLLAPTLDHVAEAVGAAAAQDCANAAYFAGGLLGALHGALICEAEGLPVAKVCAQFSELSPILGGDVAHLGKTLASGDFDHPYASLKTWSAAISRLAGHATDAGIDSRFPRFAADLFEEGVAQGFGQQEVSALIKVLRARNGAAQ

SEQ ID NO: 18 - DNA, 879 bp, Artificial Sequence
atgcgccatctgagcgtgattggcctgggcgcgatgggcgtcgcgctggcgaccaccctgctgaaggcaggacacccagtaacagtttggaatcgtagtgctgcaaaggctgctccactccaagctctaggtgctactttggctcctagtgttggagccgctatcgccgcgagcgatattaccctggtgtgcgtggataactatgcggtgagccagctgctgctggatgaagcgagcgatgcagtagccgggaagttgcttgtacaactttcgacgggaagtcctcaaggtgcacgtgcccttgagagctggagccatgcgcgcggcgcgcgctatctggatggcgcgattctgtgctttccggcgcagattggcaccagcgatgcgagcattatttgcagcggcgcgagcgcggcgtttagcgaagcggaaccggtgctgtctctcctcgctcccacactagaccacgttgccgaggctgtgggagcggccgcggctcaagactgcgcgaatgcggcgtatttcgctggaggcctgctgggcgcgctgcatggcgcgctgatttgcgaagcggaaggcctgccggtggcgaaagtgtgcgcgcagtttagcgaactgagcccgattctgggcggcgatgtggcgcatctgggcaagacattggcgagcggcgatttcgaccacccgtatgcgagcctgaagacttggagcgcggcgattagccgcctggcgggccatgcgaccgatgcgggcattgatagccgctttccgcgctttgcggcggatctgtttgaagaaggcgtggcgcagggctttggccagcaggaagtgagcgcgctgattaaagtgctgcgcgcgcgcaacggcgcggcgcagtaa

SEQ ID NO: 19 - protein, 292 aa, Artificial Sequence
MRHLSVIGLGAMGVALATTLLKAGHPVTVWNRSAAKAAPLQALGATLAPSVGAAIAASDITLVCVDNYAVSQLLLDEASDAVAGKLLVQLSTGSPQGARALESWSHARGARYLDGAILCFPAQIGTSDASIICSGASAAFSEAEPVLSLLAPTLDHVAEAVGAAAAQDCAVAAYFAGGLLGALHGALICEAEGLPVAKVCAQFSELSPTLGGDVAHLGKTLASGDFDHPYASLKTWSAAISRLAGHATDAGIDSRFPRFAADLFEEGVAQGFGQQEVSALIKVLRARNGAAQ

SEQ ID NO: 20 - DNA, 879 bp, Artificial Sequence
atgcgccatctgagcgtgattggcctgggcgcgatgggcgtcgcgctggcgaccaccctgctgaaggcaggacacccagtaacagtttggaatcgtagtgctgcaaaggctgctccactccaagctctaggtgctactttggctcctagtgttggagccgctatcgccgcgagcgatattaccctggtgtgcgtggataactatgcggtgagccagctgctgctggatgaagcgagcgatgcagtagccgggaagttgcttgtacaactttcgacgggaagtcctcaaggtgcacgtgcccttgagagctggagccatgcgcgcggcgcgcgctatctggatggcgcgattctgtgctttccggcgcagattggcaccagcgatgcgagcattatttgcagcggcgcgagcgcggcgtttagcgaagcggaaccggtgctgtctctcctcgctcccacactagaccacgttgccgaggctgtgggagcggccgcggctcaagactgcgcggtggcggcgtatttcgctggaggcctgctgggcgcgctgcatggcgcgctgatttgcgaagcggaaggcctgccggtggcgaaagtgtgcgcgcagtttagcgaactgagcccgactctgggcggcgatgtggcgcatctgggcaagacattggcgagcggcgatttcgaccacccgtatgcgagcctgaagacttggagcgcggcgattagccgcctggcgggccatgcgaccgatgcgggcattgatagccgctttccgcgctttgcggcggatctgtttgaagaaggcgtggcgcagggctttggccagcaggaagtgagcgcgctgattaaagtgctgcgcgcgcgcaacggcgcggcgcagtaa

SEQ ID NO: 21 - protein, 292 aa, Artificial Sequence
MRHLSVIGLGAMGSALATTLLKAGHPVTVWNRRAAKAAPLQALGATLAPSVGAAIAASDITLVCVDNYAVSQLLLDEASDAVAGKLLVQLSTGSPQGARALESWSHARGARYLDGAILCFPAQIGTSDASIICSGASAAFSEAEPVLSLLAPTLDHVAEAVGAAAAQDCANAAYFAGGLLGALHGALICEAEGLPVAKVCAQFSELSPILGGDVAHLGKTLASGDFDHPYASLKTWSAAISRLAGHATDAGIDSRFPRFAADLFEEGVAQGFGQQELSALIKVLRARNGAAQ

SEQ ID NO: 22 - DNA, 879 bp, Artificial Sequence; identical to SEQ ID NO: 12

SEQ ID NO: 23 - protein, 292 aa, Artificial Sequence
MRHLSVIGLGAMGSALATTLLKAGHPVTVWNRSAAKAAPLQALGATLAPSVGAAIAASDITLVCVDNYAVSQLLLDEASDAVAGKLLVQLSTGSPQGARALESWSHARGARYLDGAILCFPAQIGTSDASIICSGASAAFSEAEPVLSLLAPTLDHVAEAVGAAAAQDCASAAYFAGGLLGALHGALICEAEGLPVAKVCAQFSELSPILGGDVAHLGKTLASGDFDHPYASLKTWSAAISRLAGHATDAGIDSRFPRFAADLFEEGVAQGFGQQEVSALIKVLRARNGAAQ

SEQ ID NO: 24 - DNA, 879 bp, Artificial Sequence
atgcgccatctgagcgtgattggcctgggcgcgatgggcagcgcgctggcgaccaccctgctgaaggcaggacacccagtaacagtttggaatcgtagtgctgcaaaggctgctccactccaagctctaggtgctactttggctcctagtgttggagccgctatcgccgcgagcgatattaccctggtgtgcgtggataactatgcggtgagccagctgctgctggatgaagcgagcgatgcagtagccgggaagttgcttgtacaactttcgacgggaagtcctcaaggtgcacgtgcccttgagagctggagccatgcgcgcggcgcgcgctatctggatggcgcgattctgtgctttccggcgcagattggcaccagcgatgcgagcattatttgcagcggcgcgagcgcggcgtttagcgaagcggaaccggtgctgtctctcctcgctcccacactagaccacgttgccgaggctgtgggagcggccgcggctcaagactgcgcgagcgcggcgtatttcgctggaggcctgctgggcgcgctgcatggcgcgctgatttgcgaagcggaaggcctgccggtggcgaaagtgtgcgcgcagtttagcgaactgagcccgattctgggcggcgatgtggcgcatctgggcaagacattggcgagcggcgatttcgaccacccgtatgcgagcctgaagacttggagcgcggcgattagccgcctggcgggccatgcgaccgatgcgggcattgatagccgctttccgcgctttgcggcggatctgtttgaagaaggcgtggcgcagggctttggccagcaggaagtgagcgcgctgattaaagtgctgcgcgcgcgcaacggcgcggcgcagtaa

SEQ ID NO: 25 - protein, 292 aa, Artificial Sequence
MRHLSVIGLGAMGSALATTLLKAGHPVTVWNRSAAKAAPLQALGATLAPSVGAAIAASDITLVCVDNYAVSQLLLDEASDAVAGKLLVQLSTGSPQGARALESWSHARGARYLDGAILCFPAQIGTSDASIICSGASAAFSEAEPVLSLLAPTLDHVAEAVGAAAAQDCAAAAYFAGGLLGALHGALICEAEGLPVAKVCAQFSELSPILGGDVAHLGKTLASGDFDHPYASLKTWSAAISRLAGHATDAGIDSRFPRFAADLFEEGVAQGFGQQEVSALIKVLRARNGAAQ

SEQ ID NO: 26 - DNA, 879 bp, Artificial Sequence
atgcgccatctgagcgtgattggcctgggcgcgatgggcagcgcgctggcgaccaccctgctgaaggcaggacacccagtaacagtttggaatcgtagtgctgcaaaggctgctccactccaagctctaggtgctactttggctcctagtgttggagccgctatcgccgcgagcgatattaccctggtgtgcgtggataactatgcggtgagccagctgctgctggatgaagcgagcgatgcagtagccgggaagttgcttgtacaactttcgacgggaagtcctcaaggtgcacgtgcccttgagagctggagccatgcgcgcggcgcgcgctatctggatggcgcgattctgtgctttccggcgcagattggcaccagcgatgcgagcattatttgcagcggcgcgagcgcggcgtttagcgaagcggaaccggtgctgtctctcctcgctcccacactagaccacgttgccgaggctgtgggagcggccgcggctcaagactgcgcggcggcggcgtatttcgctggaggcctgctgggcgcgctgcatggcgcgctgatttgcgaagcggaaggcctgccggtggcgaaagtgtgcgcgcagtttagcgaactgagcccgattctgggcggcgatgtggcgcatctgggcaagacattggcgagcggcgatttcgaccacccgtatgcgagcctgaagacttggagcgcggcgattagccgcctggcgggccatgcgaccgatgcgggcattgatagccgctttccgcgctttgcggcggatctgtttgaagaaggcgtggcgcagggctttggccagcaggaagtgagcgcgctgattaaagtgctgcgcgcgcgcaacggcgcggcgcagtaa

SEQ ID NO: 27 - protein, 292 aa, Artificial Sequence
MRHLSVIGLGAMGSALATTLLKAGHPVTVWNRSAAKAAPLQALGATLAPSVGAAIAASDITLVCVDNYAVSQLLLDEASDAVAGKLLVQLSTGSPQGARALESWSHARGARYLDGAILCFPAQIGTSDASIICSGASAAFSEAEPVLSLLAPTLDHVAEAVGAAAAQDCAVVAYFAGGLLGALHGALICEAEGLPVAKVCAQFSELSPILGGDVAHLGKTLASGDFDHPYASLKTWSAAISRLAGHATDAGIDSRFPRFAADLFEEGVAQGFGQQEVSALIKVLRARNGAAQ

SEQ ID NO: 28 - DNA, 879 bp, Artificial Sequence
atgcgccatctgagcgtgattggcctgggcgcgatgggcagcgcgctggcgaccaccctgctgaaggcaggacacccagtaacagtttggaatcgtagtgctgcaaaggctgctccactccaagctctaggtgctactttggctcctagtgttggagccgctatcgccgcgagcgatattaccctggtgtgcgtggataactatgcggtgagccagctgctgctggatgaagcgagcgatgcagtagccgggaagttgcttgtacaactttcgacgggaagtcctcaaggtgcacgtgcccttgagagctggagccatgcgcgcggcgcgcgctatctggatggcgcgattctgtgctttccggcgcagattggcaccagcgatgcgagcattatttgcagcggcgcgagcgcggcgtttagcgaagcggaaccggtgctgtctctcctcgctcccacactagaccacgttgccgaggctgtgggagcggccgcggctcaagactgcgcggtggtggcgtatttcgctggaggcctgctgggcgcgctgcatggcgcgctgatttgcgaagcggaaggcctgccggtggcgaaagtgtgcgcgcagtttagcgaactgagcccgattctgggcggcgatgtggcgcatctgggcaagacattggcgagcggcgatttcgaccacccgtatgcgagcctgaagacttggagcgcggcgattagccgcctggcgggccatgcgaccgatgcgggcattgatagccgctttccgcgctttgcggcggatctgtttgaagaaggcgtggcgcagggctttggccagcaggaagtgagcgcgctgattaaagtgctgcgcgcgcgcaacggcgcggcgcagtaa

SEQ ID NO: 29 - protein, 292 aa, Artificial Sequence
MRHLSVIGLGAMGSALATTLLKAGHPVTVWNRSAAKAAPLQALGATLAPSVGAAIAASDITLVCVDNYAVSQLLLDEASDAVAGKLLVQLSTGSPQGARALESWSHARGARYLDGAILCFPAQIGTSDASIICSGASAAFSEAEPVLSLLAPTLDHVAEAVGAAAAQDCAAAAYFAGGLLGALHGALICEAEGLPVAKVCAQFSEYSPILGGDVAHLGKTLASGDFDHPGASLKLWSAAISRLAGHATDAGIDSRFPRFAADLFEEGVAQGFGQQEVSALIKVLRARNGAAQ

SEQ ID NO: 30 - DNA, 879 bp, Artificial Sequence
atgcgccatctgagcgtgattggcctgggcgcgatgggcagcgcgctggcgaccaccctgctgaaggcaggacacccagtaacagtttggaatcgtagtgctgcaaaggctgctccactccaagctctaggtgctactttggctcctagtgttggagccgctatcgccgcgagcgatattaccctggtgtgcgtggataactatgcggtgagccagctgctgctggatgaagcgagcgatgcagtagccgggaagttgcttgtacaactttcgacgggaagtcctcaaggtgcacgtgcccttgagagctggagccatgcgcgcggcgcgcgctatctggatggcgcgattctgtgctttccggcgcagattggcaccagcgatgcgagcattatttgcagcggcgcgagcgcggcgtttagcgaagcggaaccggtgctgtctctcctcgctcccacactagaccacgttgccgaggctgtgggagcggccgcggctcaagactgcgcggcggcggcgtatttcgctggaggcctgctgggcgcgctgcatggcgcgctgatttgcgaagcggaaggcctgccggtggcgaaagtgtgcgcgcagtttagcgaatatagcccgattctgggcggcgatgtggcgcatctgggcaagacattggcgagcggcgatttcgaccacccgggggcgagcctgaagctttggagcgcggcgattagccgcctggcgggccatgcgaccgatgcgggcattgatagccgctttccgcgctttgcggcggatctgtttgaagaaggcgtggcgcagggctttggccagcaggaagtgagcgcgctgattaaagtgctgcgcgcgcgcaacggcgcggcgcagtaa

SEQ ID NO: 31 - protein, 292 aa, Artificial Sequence
MRHLSVIGLGAMGSALATTLLKAGHPVTVWNRSAAKAAPLQALGATLAPSVGAAIAASDITLVCVDNYAVSQLLLDEASDAVAGKLLVQLSTGSPQGARALESWSHARGARYLDGAILCFPAQIGTSDASIICSGASAAFSEAEPVLSLLAPTLDHVAEAVGAAAAQDCAAVAYFAGGLLGALHGALICEAEGLPVAKVCAQFSELSPILGGDVAHLGKTLASGDFDHPYASLKTWSAAISRLAGHATDAGIDSRFPRFAADLFEEGVAQGFGQQEVSALIKVLRARNGAAQ

SEQ ID NO: 32 - DNA, 879 bp, Artificial Sequence
atgcgccatctgagcgtgattggcctgggcgcgatgggcagcgcgctggcgaccaccctgctgaaggcaggacacccagtaacagtttggaatcgtagtgctgcaaaggctgctccactccaagctctaggtgctactttggctcctagtgttggagccgctatcgccgcgagcgatattaccctggtgtgcgtggataactatgcggtgagccagctgctgctggatgaagcgagcgatgcagtagccgggaagttgcttgtacaactttcgacgggaagtcctcaaggtgcacgtgcccttgagagctggagccatgcgcgcggcgcgcgctatctggatggcgcgattctgtgctttccggcgcagattggcaccagcgatgcgagcattatttgcagcggcgcgagcgcggcgtttagcgaagcggaaccggtgctgtctctcctcgctcccacactagaccacgttgccgaggctgtgggagcggccgcggctcaagactgcgcggcggtggcgtatttcgctggaggcctgctgggcgcgctgcatggcgcgctgatttgcgaagcggaaggcctgccggtggcgaaagtgtgcgcgcagtttagcgaactgagcccgattctgggcggcgatgtggcgcatctgggcaagacattggcgagcggcgatttcgaccacccgtatgcgagcctgaagacttggagcgcggcgattagccgcctggcgggccatgcgaccgatgcgggcattgatagccgctttccgcgctttgcggcggatctgtttgaagaaggcgtggcgcagggctttggccagcaggaagtgagcgcgctgattaaagtgctgcgcgcgcgcaacggcgcggcgcagtaa

SEQ ID NO: 33 - protein, 292 aa, Artificial Sequence
MRHLSVIGLGAMGSALATTLLKAGHPVTVWNRSAAKAAPLQALGATLAPSVGAAIAASDITLVCVDNYAVSQLLLDEASDAVAGKLLVQLSTGSPQGARALESWSHARGARYLDGAILCFPAQIGTSDASIICSGASAAFSEAEPVLSLLAPTLDHVAEAVGAAAAQDCAAAAYFAGGLLGALHGALICEAEGLPVAKVCAQFSELSPILGGDVAHLGKTLASGDFDHPGASLKTWSAAISRLAGHATDAGIDSRFPRFAADLFEEGVAQGFGQQEVSALIKVLRARNGAAQ

SEQ ID NO: 34 - DNA, 879 bp, Artificial Sequence
atgcgccatctgagcgtgattggcctgggcgcgatgggcagcgcgctggcgaccaccctgctgaaggcaggacacccagtaacagtttggaatcgtagtgctgcaaaggctgctccactccaagctctaggtgctactttggctcctagtgttggagccgctatcgccgcgagcgatattaccctggtgtgcgtggataactatgcggtgagccagctgctgctggatgaagcgagcgatgcagtagccgggaagttgcttgtacaactttcgacgggaagtcctcaaggtgcacgtgcccttgagagctggagccatgcgcgcggcgcgcgctatctggatggcgcgattctgtgctttccggcgcagattggcaccagcgatgcgagcattatttgcagcggcgcgagcgcggcgtttagcgaagcggaaccggtgctgtctctcctcgctcccacactagaccacgttgccgaggctgtgggagcggccgcggctcaagactgcgcggcggcggcgtatttcgctggaggcctgctgggcgcgctgcatggcgcgctgatttgcgaagcggaaggcctgccggtggcgaaagtgtgcgcgcagtttagcgaactgagcccgattctgggcggcgatgtggcgcatctgggcaagacattggcgagcggcgatttcgaccacccgggcgcgagcctgaagacttggagcgcggcgattagccgcctggcgggccatgcgaccgatgcgggcattgatagccgctttccgcgctttgcggcggatctgtttgaagaaggcgtggcgcagggctttggccagcaggaagtgagcgcgctgattaaagtgctgcgcgcgcgcaacggcgcggcgcagtaa

SEQ ID NO: 35 - protein, 292 aa, Artificial Sequence
MRHLSVIGLGAMGSALATTLLKAGHPVTVWNRSAAKAAPLQALGATLAPSVGAAIAASDITLVCVDNYAVSQLLLDEASDAVAGKLLVQLSTGSPQGARALESWSHARGARYLDGAILCFPAQIGTSDASIICSGASAAFSEAEPVLSLLAPTLDHVAEAVGAAAAQDCAVVAYFAGGLLGALHGALICEAEGLPVAKVCAQFSELSPILGGDVAHLGKTLASGDFDHPGASLKTWSAAISRLAGHATDAGIDSRFPRFAADLFEEGVAQGFGQQEVSALIKVLRARNGAAQ

SEQ ID NO: 36 - DNA, 879 bp, Artificial Sequence
atgcgccatctgagcgtgattggcctgggcgcgatgggcagcgcgctggcgaccaccctgctgaaggcaggacacccagtaacagtttggaatcgtagtgctgcaaaggctgctccactccaagctctaggtgctactttggctcctagtgttggagccgctatcgccgcgagcgatattaccctggtgtgcgtggataactatgcggtgagccagctgctgctggatgaagcgagcgatgcagtagccgggaagttgcttgtacaactttcgacgggaagtcctcaaggtgcacgtgcccttgagagctggagccatgcgcgcggcgcgcgctatctggatggcgcgattctgtgctttccggcgcagattggcaccagcgatgcgagcattatttgcagcggcgcgagcgcggcgtttagcgaagcggaaccggtgctgtctctcctcgctcccacactagaccacgttgccgaggctgtgggagcggccgcggctcaagactgcgcggtggtggcgtatttcgctggaggcctgctgggcgcgctgcatggcgcgctgatttgcgaagcggaaggcctgccggtggcgaaagtgtgcgcgcagtttagcgaactgagcccgattctgggcggcgatgtggcgcatctgggcaagacattggcgagcggcgatttcgaccacccgggcgcgagcctgaagacttggagcgcggcgattagccgcctggcgggccatgcgaccgatgcgggcattgatagccgctttccgcgctttgcggcggatctgtttgaagaaggcgtggcgcagggctttggccagcaggaagtgagcgcgctgattaaagtgctgcgcgcgcgcaacggcgcggcgcagtaa

SEQ ID NO: 37 - protein, 292 aa, Artificial Sequence
MRHLSVIGLGAMGSALATTLLKAGHPVTVWNRSAAKAAPLQALGATLAPSVGAAIAASDITLVCVDNYAVSQLLLDEASDAVAGKLLVQLSTGSPQGARALESWSHARGARYLDGAILCFPAQIGTSDASIICSGASAAFSEAEPVLSLLAPTLDHVAEAVGAAAAQDCAAVAYFAGGLLGALHGALICEAEGLPVAKVCAQFSELSPILGGDVAHLGKTLASGDFDHPGASLKTWSAAISRLAGHATDAGIDSRFPRFAADLFEEGVAQGFGQQEVSALIKVLRARNGAAQ

SEQ ID NO: 38 - DNA, 879 bp, Artificial Sequence
atgcgccatctgagcgtgattggcctgggcgcgatgggcagcgcgctggcgaccaccctgctgaaggcaggacacccagtaacagtttggaatcgtagtgctgcaaaggctgctccactccaagctctaggtgctactttggctcctagtgttggagccgctatcgccgcgagcgatattaccctggtgtgcgtggataactatgcggtgagccagctgctgctggatgaagcgagcgatgcagtagccgggaagttgcttgtacaactttcgacgggaagtcctcaaggtgcacgtgcccttgagagctggagccatgcgcgcggcgcgcgctatctggatggcgcgattctgtgctttccggcgcagattggcaccagcgatgcgagcattatttgcagcggcgcgagcgcggcgtttagcgaagcggaaccggtgctgtctctcctcgctcccacactagaccacgttgccgaggctgtgggagcggccgcggctcaagactgcgcggcggttgcgtatttcgctggaggcctgctgggcgcgctgcatggcgcgctgatttgcgaagcggaaggcctgccggtggcgaaagtgtgcgcgcagtttagcgaactgagcccgattctgggcggcgatgtggcgcatctgggcaagacattggcgagcggcgatttcgaccacccgggggcgagcctgaagacttggagcgcggcgattagccgcctggcgggccatgcgaccgatgcgggcattgatagccgctttccgcgctttgcggcggatctgtttgaagaaggcgtggcgcagggctttggccagcaggaagtgagcgcgctgattaaagtgctgcgcgcgcgcaacggcgcggcgcagtaa

SEQ ID NO: 39 - protein, 292 aa, Artificial Sequence
MRHLSVIGLGAMGLALATTLLKAGHPVTVWNRGAAKAAPLQALGATLAPSVGAAIAASDITLVCVDNYAVSQLLLDEASDAVAGKLLVQLSTGSPQGARALESWSHARGARYLDGAILCFPAQIGTSDASIICSGASAAFSEAEPVLSLLAPTLDHVAEAVGAAAAQDCAVFAYFAGGLLGALHGALICEAEGLPVAKVCALFSELSPILGGDVAHLGKTLASGDFDHPYASLKTWSAAISRLAGHATDAGIDSRFPRFAADLFEEGVAQGFGQQEVSALIKVLRARNGAAQ

SEQ ID NO: 40 - DNA, 879 bp, Artificial Sequence
atgcgccatctgagcgtgattggcctgggcgcgatgggcctggcgctggcgaccaccctgctgaaggcaggacacccagtaacagtttggaatcgtggggctgcaaaggctgctccactccaagctctaggtgctactttggctcctagtgttggagccgctatcgccgcgagcgatattaccctggtgtgcgtggataactatgcggtgagccagctgctgctggatgaagcgagcgatgcagtagccgggaagttgcttgtacaactttcgacgggaagtcctcaaggtgcacgtgcccttgagagctggagccatgcgcgcggcgcgcgctatctggatggcgcgattctgtgctttccggcgcagattggcaccagcgatgcgagcattatttgcagcggcgcgagcgcggcgtttagcgaagcggaaccggtgctgtctctcctcgctcccacactagaccacgttgccgaggctgtgggagcggccgcggctcaagactgcgcggtgtttgcgtatttcgctggaggcctgctgggcgcgctgcatggcgcgctgatttgcgaagcggaaggcctgccggtggcgaaagtgtgcgcgctttttagcgaactgagcccgattctgggcggcgatgtggcgcatctgggcaagacattggcgagcggcgatttcgaccacccgtatgcgagcctgaagacttggagcgcggcgattagccgcctggcgggccatgcgaccgatgcgggcattgatagccgctttccgcgctttgcggcggatctgtttgaagaaggcgtggcgcagggctttggccagcaggaagtgagcgcgctgattaaagtgctgcgcgcgcgcaacggcgcggcgcagtaa

SEQ ID NO: 41 - protein, 292 aa, Artificial Sequence
MRHLSVIGLGAMGQALATTLLKAGHPVTVWNRSAAKAAPLQALGATLAPSVGAAIAASDITLVCVDNYAVSQLLLDEASDAVAGKLLVQLSTGSPQGARALESWSHARGARYLDGAILCFPAQIGTSDASIICSGASAAFSEAEPVLSLLAPTLDHVAEAVGAAAAQDCAAVAYFAGGLLGALHGALICEAEGLPVAKVCAQFSELSPILGGDVAHLGKTLASGDFDHPGASLKTWSAAISRLAGHATDAGIDSRFPRFAADLFEEGVAQGFGQQEVSALIKVLRARNGAAQ

SEQ ID NO: 42 - DNA, 879 bp, Artificial Sequence
atgcgccatctgagcgtgattggcctgggcgcgatgggccaggcgctggcgaccaccctgctgaaggcaggacacccagtaacagtttggaatcgtagtgctgcaaaggctgctccactccaagctctaggtgctactttggctcctagtgttggagccgctatcgccgcgagcgatattaccctggtgtgcgtggataactatgcggtgagccagctgctgctggatgaagcgagcgatgcagtagccgggaagttgcttgtacaactttcgacgggaagtcctcaaggtgcacgtgcccttgagagctggagccatgcgcgcggcgcgcgctatctggatggcgcgattctgtgctttccggcgcagattggcaccagcgatgcgagcattatttgcagcggcgcgagcgcggcgtttagcgaagcggaaccggtgctgtctctcctcgctcccacactagaccacgttgccgaggctgtgggagcggccgcggctcaagactgcgcggcggttgcgtatttcgctggaggcctgctgggcgcgctgcatggcgcgctgatttgcgaagcggaaggcctgccggtggcgaaagtgtgcgcgcagtttagcgaactgagcccgattctgggcggcgatgtggcgcatctgggcaagacattggcgagcggcgatttcgaccacccgggggcgagcctgaagacttggagcgcggcgattagccgcctggcgggccatgcgaccgatgcgggcattgatagccgctttccgcgctttgcggcggatctgtttgaagaaggcgtggcgcagggctttggccagcaggaagtgagcgcgctgattaaagtgctgcgcgcgcgcaacggcgcggcgcagtaa

SEQ ID NO: 43 - protein, 292 aa, Artificial Sequence
MRHLSVIGLGAMGVALATTLLKAGHPVTVWNRDAAKAAPLQALGATLAPSVGAAIAASDITLVCVDNYAVSQLLLDEASDAVAGKLLVQLSTGSPQGARALESWSHARGARYLDGAILTFPAQIGTSDASIICSGASAAFSEAEPVLSLLAPTLDHVAEAVGAAAAQDCAAFAYFAGGLLGALHGALICEAEGLPVAKVCAQFSELSPILGGDVAHLGKTLASGDFDHPAASLKTWSAYISRLAGHATDAGIDSRFPRFAADLFEEGVAQGFGQQEVSALIKVLRARNGAAQ

SEQ ID NO: 44 - DNA, 879 bp, Artificial Sequence
atgcgccatctgagcgtgattggcctgggcgcgatgggcgttgcgctggcgaccaccctgctgaaggcaggacacccagtaacagtttggaatcgtgatgctgcaaaggctgctccactccaagctctaggtgctactttggctcctagtgttggagccgctatcgccgcgagcgatattaccctggtgtgcgtggataactatgcggtgagccagctgctgctggatgaagcgagcgatgcagtagccgggaagttgcttgtacaactttcgacgggaagtcctcaaggtgcacgtgcccttgagagctggagccatgcgcgcggcgcgcgctatctggatggcgcgattctgacttttccggcgcagattggcaccagcgatgcgagcattatttgcagcggcgcgagcgcggcgtttagcgaagcggaaccggtgctgtctctcctcgctcccacactagaccacgttgccgaggctgtgggagcggccgcggctcaagactgcgcggcgtttgcgtatttcgctggaggcctgctgggcgcgctgcatggcgcgctgatttgcgaagcggaaggcctgccggtggcgaaagtgtgcgcgcagtttagcgaactgagcccgattctgggcggcgatgtggcgcatctgggcaagacattggcgagcggcgatttcgaccacccggctgcgagcctgaagacttggagcgcgtatattagccgcctggcgggccatgcgaccgatgcgggcattgatagccgctttccgcgctttgcggcggatctgtttgaagaaggcgtggcgcagggctttggccagcaggaagtgagcgcgctgattaaagtgctgcgcgcgcgcaacggcgcggcgcagtaa

SEQ ID NO: 45 - protein, 292 aa, Artificial Sequence
MRHLSVIGLGAMGVALATTLLKAGHPVTVWNRSAAKAAPLQALGATLAPSVGAAIAASDITLVCVDNYAVSQLLLDEASDAVAGKLLVQLSTGSPQGARALESWSHARGARYLDGAILTFPAQIGTSDASIICSGASAAFSEAEPVLSLLAPTLDHVAEAVGAAAAQDCAAFAYFAGGLLGALHGALICEAEGLPVAKVCAQFSELSPILGGDVAHLGKTLASGDFDHPGASLKLWSAAISRLAGHATDAGIDSRFPRFAADLFEEGVAQGFGQQEVSALIKVLRARNGAAQ

SEQ ID NO: 46 - DNA, 879 bp, Artificial Sequence
atgcgccatctgagcgtgattggcctgggcgcgatgggcgttgcgctggcgaccaccctgctgaaggcaggacacccagtaacagtttggaatcgtagtgctgcaaaggctgctccactccaagctctaggtgctactttggctcctagtgttggagccgctatcgccgcgagcgatattaccctggtgtgcgtggataactatgcggtgagccagctgctgctggatgaagcgagcgatgcagtagccgggaagttgcttgtacaactttcgacgggaagtcctcaaggtgcacgtgcccttgagagctggagccatgcgcgcggcgcgcgctatctggatggcgcgattctgacttttccggcgcagattggcaccagcgatgcgagcattatttgcagcggcgcgagcgcggcgtttagcgaagcggaaccggtgctgtctctcctcgctcccacactagaccacgttgccgaggctgtgggagcggccgcggctcaagactgcgcggcgtttgcgtatttcgctggaggcctgctgggcgcgctgcatggcgcgctgatttgcgaagcggaaggcctgccggtggcgaaagtgtgcgcgcagtttagcgaactgagcccgattctgggcggcgatgtggcgcatctgggcaagacattggcgagcggcgatttcgaccacccgggggcgagcctgaagctttggagcgcggcgattagccgcctggcgggccatgcgaccgatgcgggcattgatagccgctttccgcgctttgcggcggatctgtttgaagaaggcgtggcgcagggctttggccagcaggaagtgagcgcgctgattaaagtgctgcgcgcgcgcaacggcgcggcgcagtaa

SEQ ID NO: 47 - protein, 292 aa, Artificial Sequence
MRHLSVIGLGAMGSALATTLLKAGHPVTVWNRGAAKAAPLQALGATLAPSVGAAIAASDITLVCVDNYAVSQLLLDEASDAVAGKLLVQLSTGSPQGARALESWSHARGARYLDGAILCFPAQIGTSDATIICSGASAAFSEAEPVLSLLAPTLDHVAEAVGAAAAQDCAAVAYFAGGLLGALHGALICEAEGLPVAKVCAQFSELSPILGGDVAHLGKTLASGDFDHPGASLKTWSAAISRLAGHATDAGIDSRFPRFAADLFEEGVAQGFGQQEVSALIKVLRARNGAAQ

SEQ ID NO: 48 - DNA, 879 bp, Artificial Sequence
atgcgccatctgagcgtgattggcctgggcgcgatgggcagcgcgctggcgaccaccctgctgaaggcaggacacccagtaacagtttggaatcgtggggctgcaaaggctgctccactccaagctctaggtgctactttggctcctagtgttggagccgctatcgccgcgagcgatattaccctggtgtgcgtggataactatgcggtgagccagctgctgctggatgaagcgagcgatgcagtagccgggaagttgcttgtacaactttcgacgggaagtcctcaaggtgcacgtgcccttgagagctggagccatgcgcgcggcgcgcgctatctggatggcgcgattctgtgctttccggcgcagattggcaccagcgatgcgactattatttgcagcggcgcgagcgcggcgtttagcgaagcggaaccggtgctgtctctcctcgctcccacactagaccacgttgccgaggctgtgggagcggccgcggctcaagactgcgcggcggttgcgtatttcgctggaggcctgctgggcgcgctgcatggcgcgctgatttgcgaagcggaaggcctgccggtggcgaaagtgtgcgcgcagtttagcgaactgagcccgattctgggcggcgatgtggcgcatctgggcaagacattggcgagcggcgatttcgaccacccgggggcgagcctgaagacttggagcgcggcgattagccgcctggcgggccatgcgaccgatgcgggcattgatagccgctttccgcgctttgcggcggatctgtttgaagaaggcgtggcgcagggctttggccagcaggaagtgagcgcgctgattaaagtgctgcgcgcgcgcaacggcgcggcgcagtaa

SEQ ID NO: 49 - protein, 292 aa, Artificial Sequence
MRHLSVIGLGAMGQALATTLLKAGHPVTVWNRSAAKAAPLQALGATLAPSVGAAIAASDITLVCVDNYAVSQLLLDEASDAVAGKLLVQLSTGSPQGARALESWSHARGARYLDGAIVCFPAQIGTSDASIICSGASAAFSEAEPVLSLLAPTLDHVAEAVGAAAAQDCAAVAYFAGGLLGALHGALICEAEGLPVAKVCALFSELSPILGGDVAHLGKTLASGDFDHPAASLKTWSAAISRLAGHATDAGIDSRFPRFAADLFEEGVAQGFGQQEVSALIKVLRARNGAAQ

SEQ ID NO: 50 - DNA, 879 bp, Artificial Sequence
atgcgccatctgagcgtgattggcctgggcgcgatgggccaggcgctggcgaccaccctgctgaaggcaggacacccagtaacagtttggaatcgtagtgctgcaaaggctgctccactccaagctctaggtgctactttggctcctagtgttggagccgctatcgccgcgagcgatattaccctggtgtgcgtggataactatgcggtgagccagctgctgctggatgaagcgagcgatgcagtagccgggaagttgcttgtacaactttcgacgggaagtcctcaaggtgcacgtgcccttgagagctggagccatgcgcgcggcgcgcgctatctggatggcgcgattgtttgctttccggcgcagattggcaccagcgatgcgagcattatttgcagcggcgcgagcgcggcgtttagcgaagcggaaccggtgctgtctctcctcgctcccacactagaccacgttgccgaggctgtgggagcggccgcggctcaagactgcgcggcggttgcgtatttcgctggaggcctgctgggcgcgctgcatggcgcgctgatttgcgaagcggaaggcctgccggtggcgaaagtgtgcgcgctttttagcgaactgagcccgattctgggcggcgatgtggcgcatctgggcaagacattggcgagcggcgatttcgaccacccggctgcgagcctgaagacttggagcgcggcgattagccgcctggcgggccatgcgaccgatgcgggcattgatagccgctttccgcgctttgcggcggatctgtttgaagaaggcgtggcgcagggctttggccagcaggaagtgagcgcgctgattaaagtgctgcgcgcgcgcaacggcgcggcgcagtaa

SEQ ID NO: 51 - protein, 292 aa, Artificial Sequence
MRHLSVIGLGAMGQALATTLLKAGHPVTVWNRLAAKAAPLQALGATLAPSVGAAIAASDITLVCVDNYAVSQLLLDEASDAVAGKLLVQLSTGSPQGARALESWSHARGARYLDGAIVCFPAQIGTSDASIICSGASAAFSEAEPVLSLLAPTLDHVAEAVGAAAAQDCAAVAYFAGGLLGALHGALICEAEGLPVAKVCALFSELSPILGGDVAHLGKTLASGDFDHPLASLKTWSAAISRLAGHATDAGIDSRFPRFAADLFEEGVAQGFGQQEVSALIKVLRARNGAAQ

SEQ ID NO: 52 - DNA, 879 bp, Artificial Sequence
atgcgccatctgagcgtgattggcctgggcgcgatgggccaggcgctggcgaccaccctgctgaaggcaggacacccagtaacagtttggaatcgtcttgctgcaaaggctgctccactccaagctctaggtgctactttggctcctagtgttggagccgctatcgccgcgagcgatattaccctggtgtgcgtggataactatgcggtgagccagctgctgctggatgaagcgagcgatgcagtagccgggaagttgcttgtacaactttcgacgggaagtcctcaaggtgcacgtgcccttgagagctggagccatgcgcgcggcgcgcgctatctggatggcgcgattgtttgctttccggcgcagattggcaccagcgatgcgagcattatttgcagcggcgcgagcgcggcgtttagcgaagcggaaccggtgctgtctctcctcgctcccacactagaccacgttgccgaggctgtgggagcggccgcggctcaagactgcgcggcggttgcgtatttcgctggaggcctgctgggcgcgctgcatggcgcgctgatttgcgaagcggaaggcctgccggtggcgaaagtgtgcgcgctttttagcgaactgagcccgattctgggcggcgatgtggcgcatctgggcaagacattggcgagcggcgatttcgaccacccgctggcgagcctgaagacttggagcgcggcgattagccgcctggcgggccatgcgaccgatgcgggcattgatagccgctttccgcgctttgcggcggatctgtttgaagaaggcgtggcgcagggctttggccagcaggaagtgagcgcgctgattaaagtgctgcgcgcgcgcaacggcgcggcgcagtaa

SEQ ID NO: 53 - protein, 292 aa, Artificial Sequence
MRHLSVIGLGAMGQALATTLLKAGHPVTVWNRGAAKAAPLQALGATLAPSVGAAIAASDITLVCVDNYAVSQLLLDEASDAVAGKLLVQLSTGSPQGARALESWSHARGARYLDGAILDFPAQIGTSDATIICSGASAAFSEAEPVLSLLAPTLDHVAEAVGAAAAQDCAAFAYFAGGLLGALHGALICEAEGLPVAKVCAAFSELSPILGGDVAHLGKTLASGDFDHPGASLKTWSAAISRLAGHATDAGIDSRFPRFAADLFEEGVAQGFGQQEVSALIKVLRARNGAAQ

SEQ ID NO: 54 - DNA, 879 bp, Artificial Sequence
atgcgccatctgagcgtgattggcctgggcgcgatgggccaggcgctggcgaccaccctgctgaaggcaggacacccagtaacagtttggaatcgtggggctgcaaaggctgctccactccaagctctaggtgctactttggctcctagtgttggagccgctatcgccgcgagcgatattaccctggtgtgcgtggataactatgcggtgagccagctgctgctggatgaagcgagcgatgcagtagccgggaagttgcttgtacaactttcgacgggaagtcctcaaggtgcacgtgcccttgagagctggagccatgcgcgcggcgcgcgctatctggatggcgcgattctggattttccggcgcagattggcaccagcgatgcgactattatttgcagcggcgcgagcgcggcgtttagcgaagcggaaccggtgctgtctctcctcgctcccacactagaccacgttgccgaggctgtgggagcggccgcggctcaagactgcgcggcgtttgcgtatttcgctggaggcctgctgggcgcgctgcatggcgcgctgatttgcgaagcggaaggcctgccggtggcgaaagtgtgcgcggcttttagcgaactgagcccgattctgggcggcgatgtggcgcatctgggcaagacattggcgagcggcgatttcgaccacccgggggcgagcctgaagacttggagcgcggcgattagccgcctggcgggccatgcgaccgatgcgggcattgatagccgctttccgcgctttgcggcggatctgtttgaagaaggcgtggcgcagggctttggccagcaggaagtgagcgcgctgattaaagtgctgcgcgcgcgcaacggcgcggcgcagtaa

SEQ ID NO: 55 - protein, 292 aa, Artificial Sequence
MRHLSVIGLGAMGQALATTLLKAGHPVTVWNRAAAKAAPLQALGATLAPSVGAAIAASDITLVCVDNYAVSQLLLDEASDAVAGKLLVQLSTGSPQGARALESWSHARGARYLDGAILCFPAQIGTSDASIICSGASAAFSEAEPVLSLLAPTLDHVAEAVGAAAAQDCAAVAYFAGGLLGALHGALICEAEGLPVAKVCAQFSEFSPILGGDVAHLGKTLASGDFDHPGASLKTWSALISRLAGHATDAGIDSRFPRFAADLFEEGVAQGFGQQEVSALIKVLRARNGAAQ

SEQ ID NO: 56 - DNA, 879 bp, Artificial Sequence
atgcgccatctgagcgtgattggcctgggcgcgatgggccaggcgctggcgaccaccctgctgaaggcaggacacccagtaacagtttggaatcgtgcggctgcaaaggctgctccactccaagctctaggtgctactttggctcctagtgttggagccgctatcgccgcgagcgatattaccctggtgtgcgtggataactatgcggtgagccagctgctgctggatgaagcgagcgatgcagtagccgggaagttgcttgtacaactttcgacgggaagtcctcaaggtgcacgtgcccttgagagctggagccatgcgcgcggcgcgcgctatctggatggcgcgattctgtgctttccggcgcagattggcaccagcgatgcgagcattatttgcagcggcgcgagcgcggcgtttagcgaagcggaaccggtgctgtctctcctcgctcccacactagaccacgttgccgaggctgtgggagcggccgcggctcaagactgcgcggcggttgcgtatttcgctggaggcctgctgggcgcgctgcatggcgcgctgatttgcgaagcggaaggcctgccggtggcgaaagtgtgcgcgcagtttagcgaatttagcccgattctgggcggcgatgtggcgcatctgggcaagacattggcgagcggcgatttcgaccacccgggggcgagcctgaagacttggagcgcgctgattagccgcctggcgggccatgcgaccgatgcgggcattgatagccgctttccgcgctttgcggcggatctgtttgaagaaggcgtggcgcagggctttggccagcaggaagtgagcgcgctgattaaagtgctgcgcgcgcgcaacggcgcggcgcagtaa

SEQ ID NO: 57 - protein, 292 aa, Artificial Sequence
MRHLSVIGLGAMGQALATTLLKAGHPVTVWNRAAAKAAPLQALGATLAPSVGAAIAASDITLVCVDNYAVSQLLLDEASDAVAGKLLVQLSTGSPQGARALESWSHARGARYLDGAIVCFPAQIGTSDASIICSGASAAFSEAEPVLSLLAPTLDHVAEAVGAAAAQDCAAVAYFAGGLLGALHGALICEAEGLPVAKVCAQFSELSPILGGDVAHLGKTLASGDFDHPGASLKTWSAAISRLAGHATDAGIDSRFPRFAADLFEEGVAQGFGQQEVSALIKVLRARNGAAQ

SEQ ID NO: 58 - DNA, 879 bp, Artificial Sequence
atgcgccatctgagcgtgattggcctgggcgcgatgggccaggcgctggcgaccaccctgctgaaggcaggacacccagtaacagtttggaatcgtgcggctgcaaaggctgctccactccaagctctaggtgctactttggctcctagtgttggagccgctatcgccgcgagcgatattaccctggtgtgcgtggataactatgcggtgagccagctgctgctggatgaagcgagcgatgcagtagccgggaagttgcttgtacaactttcgacgggaagtcctcaaggtgcacgtgcccttgagagctggagccatgcgcgcggcgcgcgctatctggatggcgcgattgtttgctttccggcgcagattggcaccagcgatgcgagcattatttgcagcggcgcgagcgcggcgtttagcgaagcggaaccggtgctgtctctcctcgctcccacactagaccacgttgccgaggctgtgggagcggccgcggctcaagactgcgcggcggttgcgtatttcgctggaggcctgctgggcgcgctgcatggcgcgctgatttgcgaagcggaaggcctgccggtggcgaaagtgtgcgcgcagtttagcgaactgagcccgattctgggcggcgatgtggcgcatctgggcaagacattggcgagcggcgatttcgaccacccgggggcgagcctgaagacttggagcgcggcgattagccgcctggcgggccatgcgaccgatgcgggcattgatagccgctttccgcgctttgcggcggatctgtttgaagaaggcgtggcgcagggctttggccagcaggaagtgagcgcgctgattaaagtgctgcgcgcgcgcaacggcgcggcgcagtaa

SEQ ID NO: 59 - protein, 292 aa, Artificial Sequence
MRHLSVIGLGAMGVALATTLLKAGHPVTVWNRGAAKAAPLQALGATLAPSVGAAIAASDITLVCVDNYAVSQLLLDEASDAVAGKLLVQLSTGSPQGARALESWSHARGARYLDGAILCFPAQIGTSDATIICSGASAAFSEAEPVLSLLAPTLDHVAEAVGAAAAQDCAAVAYFAGGLLGALHGALICEAEGLPVAKVCAQFSELSPLLGGDVAHLGKTLASGDFDHPGASLKTWSAAISRLAGHATDAGIDSRFPRFAADLFEEGVAQGFGQQEVSALIKVLRARNGAAQ

SEQ ID NO: 60 - DNA, 879 bp, Artificial Sequence
atgcgccatctgagcgtgattggcctgggcgcgatgggcgttgcgctggcgaccaccctgctgaaggcaggacacccagtaacagtttggaatcgtggggctgcaaaggctgctccactccaagctctaggtgctactttggctcctagtgttggagccgctatcgccgcgagcgatattaccctggtgtgcgtggataactatgcggtgagccagctgctgctggatgaagcgagcgatgcagtagccgggaagttgcttgtacaactttcgacgggaagtcctcaaggtgcacgtgcccttgagagctggagccatgcgcgcggcgcgcgctatctggatggcgcgattctgtgctttccggcgcagattggcaccagcgatgcgactattatttgcagcggcgcgagcgcggcgtttagcgaagcggaaccggtgctgtctctcctcgctcccacactagaccacgttgccgaggctgtgggagcggccgcggctcaagactgcgcggcggttgcgtatttcgctggaggcctgctgggcgcgctgcatggcgcgctgatttgcgaagcggaaggcctgccggtggcgaaagtgtgcgcgcagtttagcgaactgagcccgctgctgggcggcgatgtggcgcatctgggcaagacattggcgagcggcgatttcgaccacccgggggcgagcctgaagacttggagcgcggcgattagccgcctggcgggccatgcgaccgatgcgggcattgatagccgctttccgcgctttgcggcggatctgtttgaagaaggcgtggcgcagggctttggccagcaggaagtgagcgcgctgattaaagtgctgcgcgcgcgcaacggcgcggcgcagtaa

SEQ ID NO: 61 - protein, 292 aa, Artificial Sequence
MRHLSVIGLGAMGSALATTLLKAGHPVTVWNRGAAKAAPLQALGATLAPSVGAAIAASDITLVCVDNYAVSQLLLDEASDAVAGKLLVQLSTGSPQGARALESWSHARGARYLDGAIVCFPAQIGTSDATIICSGASAAFSEAEPVLSLLAPTLDHVAEAVGAAAAQDCAAVAYFAGGLLGALHGALICEAEGLPVAKVCAQFSELSPILGGDVAHLGKTLASGDFDHPGASLLTWSAAISRLAGHATDAGIDSRFPRFAADLFEEGVAQGFGQQEVSALIKVLRARNGAAQ

SEQ ID NO: 62 - DNA, 879 bp, Artificial Sequence
atgcgccatctgagcgtgattggcctgggcgcgatgggcagcgcgctggcgaccaccctgctgaaggcaggacacccagtaacagtttggaatcgtggggctgcaaaggctgctccactccaagctctaggtgctactttggctcctagtgttggagccgctatcgccgcgagcgatattaccctggtgtgcgtggataactatgcggtgagccagctgctgctggatgaagcgagcgatgcagtagccgggaagttgcttgtacaactttcgacgggaagtcctcaaggtgcacgtgcccttgagagctggagccatgcgcgcggcgcgcgctatctggatggcgcgattgtttgctttccggcgcagattggcaccagcgatgcgactattatttgcagcggcgcgagcgcggcgtttagcgaagcggaaccggtgctgtctctcctcgctcccacactagaccacgttgccgaggctgtgggagcggccgcggctcaagactgcgcggcggttgcgtatttcgctggaggcctgctgggcgcgctgcatggcgcgctgatttgcgaagcggaaggcctgccggtggcgaaagtgtgcgcgcagtttagcgaactgagcccgattctgggcggcgatgtggcgcatctgggcaagacattggcgagcggcgatttcgaccacccgggggcgagcctgctgacttggagcgcggcgattagccgcctggcgggccatgcgaccgatgcgggcattgatagccgctttccgcgctttgcggcggatctgtttgaagaaggcgtggcgcagggctttggccagcaggaagtgagcgcgctgattaaagtgctgcgcgcgcgcaacggcgcggcgcagtaa

SEQ ID NO: 63 - protein, 292 aa, Artificial Sequence
MRHLSVIGLGAMGSALATTLLKAGHPVTVWNRGAAKAAPLQALGATLAPSVGAAIAASDITLVCVDNYAVSQLLLDEASDAVAGKLLVQLSTGSPQGARALESWSHARGARYLDGAILDFPAQIGTSDATIICSGASAAFSEAEPVLSLLAPTLDHVAEAVGAAAAQDCAAVAYFAGGLLGALHGALICEAEGLPVAKVCAAFSELSPILGGDVAHLGKTLASGDFDHPGASLKTWSAYISRLAGHATDAGIDSRFPRFAADLFEEGVAQGFGQQEVSALIKVLRARNGAAQ

SEQ ID NO: 64 - DNA, 879 bp, Artificial Sequence
atgcgccatctgagcgtgattggcctgggcgcgatgggcagcgcgctggcgaccaccctgctgaaggcaggacacccagtaacagtttggaatcgtggggctgcaaaggctgctccactccaagctctaggtgctactttggctcctagtgttggagccgctatcgccgcgagcgatattaccctggtgtgcgtggataactatgcggtgagccagctgctgctggatgaagcgagcgatgcagtagccgggaagttgcttgtacaactttcgacgggaagtcctcaaggtgcacgtgcccttgagagctggagccatgcgcgcggcgcgcgctatctggatggcgcgattctggattttccggcgcagattggcaccagcgatgcgactattatttgcagcggcgcgagcgcggcgtttagcgaagcggaaccggtgctgtctctcctcgctcccacactagaccacgttgccgaggctgtgggagcggccgcggctcaagactgcgcggcggttgcgtatttcgctggaggcctgctgggcgcgctgcatggcgcgctgatttgcgaagcggaaggcctgccggtggcgaaagtgtgcgcggcgtttagcgaactgagcccgattctgggcggcgatgtggcgcatctgggcaagacattggcgagcggcgatttcgaccacccgggggcgagcctgaagacttggagcgcgtatattagccgcctggcgggccatgcgaccgatgcgggcattgatagccgctttccgcgctttgcggcggatctgtttgaagaaggcgtggcgcagggctttggccagcaggaagtgagcgcgctgattaaagtgctgcgcgcgcgcaacggcgcggcgcagtaa

SEQ ID NO: 65 - protein, 292 aa, Artificial Sequence
MRHLSVIGLGAMGQALATTLLKAGHPVTVWNRDAAKAAPLQALGATLAPSVGAAIAASDITLVCVDNYAVSQLLLDEASDAVAGKLLVQLSTGSPQGARALESWSHARGARYLDGAILCFPAQIGTSDATIICSGASAAFSEAEPVLSLLAPTLDHVAEAVGAAAAQDCAAVAYFAGGLLGALHGALICEAEGLPVAKVCAQFSELSPILGGDVAHLGKTLASGDFDHPGASLLTWSAAISRLAGHATDAGIDSRFPRFAADLFEEGVAQGFGQQEVSALIKVLRARNGAAQ

SEQ ID NO: 66 - DNA, 879 bp, Artificial Sequence
atgcgccatctgagcgtgattggcctgggcgcgatgggccaggcgctggcgaccaccctgctgaaggcaggacacccagtaacagtttggaatcgtgatgctgcaaaggctgctccactccaagctctaggtgctactttggctcctagtgttggagccgctatcgccgcgagcgatattaccctggtgtgcgtggataactatgcggtgagccagctgctgctggatgaagcgagcgatgcagtagccgggaagttgcttgtacaactttcgacgggaagtcctcaaggtgcacgtgcccttgagagctggagccatgcgcgcggcgcgcgctatctggatggcgcgattctgtgctttccggcgcagattggcaccagcgatgcgactattatttgcagcggcgcgagcgcggcgtttagcgaagcggaaccggtgctgtctctcctcgctcccacactagaccacgttgccgaggctgtgggagcggccgcggctcaagactgcgcggcggttgcgtatttcgctggaggcctgctgggcgcgctgcatggcgcgctgatttgcgaagcggaaggcctgccggtggcgaaagtgtgcgcgcagtttagcgaactgagcccgattctgggcggcgatgtggcgcatctgggcaagacattggcgagcggcgatttcgaccacccgggggcgagcctgctgacttggagcgcggcgattagccgcctggcgggccatgcgaccgatgcgggcattgatagccgctttccgcgctttgcggcggatctgtttgaagaaggcgtggcgcagggctttggccagcaggaagtgagcgcgctgattaaagtgctgcgcgcgcgcaacggcgcggcgcagtaa

SEQ ID NO: 67 - protein, 292 aa, Artificial Sequence
MRHLSVIGLGAMGVALATTLLKAGHPVTVWNRGAAKAAPLQALGATLAPSVGAAIAASDITLVCVDNYAVSQLLLDEASDAVAGKLLVQLSTGSPQGARALESWSHARGARYLDGAILTFPAQIGTSDATIICSGASAAFSEAEPVLSLLAPTLDHVAEAVGAAAAQDCAAFAYFAGGLLGALHGALICEAEGLPVAKVCAQFSELSPILGGDVAHLGKTLASGDFDHPGASLKLWSAAISRLAGHATDAGIDSRFPRFAADLFEEGVAQGFGQQEVSALIKVLRARNGAAQ

SEQ ID NO: 68 - DNA, 879 bp, Artificial Sequence
atgcgccatctgagcgtgattggcctgggcgcgatgggcgttgcgctggcgaccaccctgctgaaggcaggacacccagtaacagtttggaatcgtggggctgcaaaggctgctccactccaagctctaggtgctactttggctcctagtgttggagccgctatcgccgcgagcgatattaccctggtgtgcgtggataactatgcggtgagccagctgctgctggatgaagcgagcgatgcagtagccgggaagttgcttgtacaactttcgacgggaagtcctcaaggtgcacgtgcccttgagagctggagccatgcgcgcggcgcgcgctatctggatggcgcgattctgacttttccggcgcagattggcaccagcgatgcgactattatttgcagcggcgcgagcgcggcgtttagcgaagcggaaccggtgctgtctctcctcgctcccacactagaccacgttgccgaggctgtgggagcggccgcggctcaagactgcgcggcgtttgcgtatttcgctggaggcctgctgggcgcgctgcatggcgcgctgatttgcgaagcggaaggcctgccggtggcgaaagtgtgcgcgcagtttagcgaactgagcccgattctgggcggcgatgtggcgcatctgggcaagacattggcgagcggcgatttcgaccacccgggggcgagcctgaagctgtggagcgcggcgattagccgcctggcgggccatgcgaccgatgcgggcattgatagccgctttccgcgctttgcggcggatctgtttgaagaaggcgtggcgcagggctttggccagcaggaagtgagcgcgctgattaaagtgctgcgcgcgcgcaacggcgcggcgcagtaa

SEQ ID NO: 69 - protein, 292 aa, Artificial Sequence
MRHLSVIGLGAMGVALATTLLKAGHPVTVWNRDAAKAAPLQALGATLAPSVGAAIAASDITLVCVDNYAVSQLLLDEASDAVAGKLLVQLSTGSPQGARALESWSHARGARYLDGAILTFPAQIGTSDACIICSGASAAFSEAEPVLSLLAPTLDHVAEAVGAAAAQDCAAFAYFAGGLLGALHGALICEAEGLPVAKVCAQFSELSPILGGDVAHLGKTLASGDFDHPGASLKTWSAYISRLAGHATDAGIDSRFPRFAADLFEEGVAQGFGQQEVSALIKVLRARNGAAQ

SEQ ID NO: 70 - DNA, 879 bp, Artificial Sequence
atgcgccatctgagcgtgattggcctgggcgcgatgggcgttgcgctggcgaccaccctgctgaaggcaggacacccagtaacagtttggaatcgtgatgctgcaaaggctgctccactccaagctctaggtgctactttggctcctagtgttggagccgctatcgccgcgagcgatattaccctggtgtgcgtggataactatgcggtgagccagctgctgctggatgaagcgagcgatgcagtagccgggaagttgcttgtacaactttcgacgggaagtcctcaaggtgcacgtgcccttgagagctggagccatgcgcgcggcgcgcgctatctggatggcgcgattctgacttttccggcgcagattggcaccagcgatgcgtgtattatttgcagcggcgcgagcgcggcgtttagcgaagcggaaccggtgctgtctctcctcgctcccacactagaccacgttgccgaggctgtgggagcggccgcggctcaagactgcgcggcgtttgcgtatttcgctggaggcctgctgggcgcgctgcatggcgcgctgatttgcgaagcggaaggcctgccggtggcgaaagtgtgcgcgcagtttagcgaactgagcccgattctgggcggcgatgtggcgcatctgggcaagacattggcgagcggcgatttcgaccacccgggggcgagcctgaagacttggagcgcgtatattagccgcctggcgggccatgcgaccgatgcgggcattgatagccgctttccgcgctttgcggcggatctgtttgaagaaggcgtggcgcagggctttggccagcaggaagtgagcgcgctgattaaagtgctgcgcgcgcgcaacggcgcggcgcagtaa

SEQ ID NO: 71 - protein, 292 aa, Artificial Sequence
MRHLSVIGLGAMGQALATTLLKAGHPVTVWNRQAAKAAPLQALGATLAPSVGAAIAASDITLVCVDNYAVSQLLLDEASDAVAGKLLVQLSTGSPQGARALESWSHARGARYLDGAIVCFPAQIGTSDATIICSGASAAFSEAEPVLSLLAPTLDHVAEAVGAAAAQDCAAVAYFAGGLLGALHGALICEAEGLPVAKVCAQFSEYSPLLGGDVAHLGKTLASGDFDHPGASLKTWSAAISRLAGHATDAGIDSRFPRFAADLFEEGVAQGFGQQEVSALIKVLRARNGAAQ

SEQ ID NO: 72 - DNA, 879 bp, Artificial Sequence
atgcgccatctgagcgtgattggcctgggcgcgatgggccaggcgctggcgaccaccctgctgaaggcaggacacccagtaacagtttggaatcgtcaggctgcaaaggctgctccactccaagctctaggtgctactttggctcctagtgttggagccgctatcgccgcgagcgatattaccctggtgtgcgtggataactatgcggtgagccagctgctgctggatgaagcgagcgatgcagtagccgggaagttgcttgtacaactttcgacgggaagtcctcaaggtgcacgtgcccttgagagctggagccatgcgcgcggcgcgcgctatctggatggcgcgattgtttgctttccggcgcagattggcaccagcgatgcgactattatttgcagcggcgcgagcgcggcgtttagcgaagcggaaccggtgctgtctctcctcgctcccacactagaccacgttgccgaggctgtgggagcggccgcggctcaagactgcgcggcggttgcgtatttcgctggaggcctgctgggcgcgctgcatggcgcgctgatttgcgaagcggaaggcctgccggtggcgaaagtgtgcgcgcagtttagcgaatatagcccgctgctgggcggcgatgtggcgcatctgggcaagacattggcgagcggcgatttcgaccacccgggggcgagcctgaagacttggagcgcggcgattagccgcctggcgggccatgcgaccgatgcgggcattgatagccgctttccgcgctttgcggcggatctgtttgaagaaggcgtggcgcagggctttggccagcaggaagtgagcgcgctgattaaagtgctgcgcgcgcgcaacggcgcggcgcagtaa

SEQ ID NO: 73 - protein, 292 aa, Artificial Sequence
MRHLSVIGLGAMGQALATTLLKAGHPVTVWNRGAAKAAPLQALGATLAPSVGAAIAASDITLVCVDNYAVSQLLLDEASDAVAGKLLVQLSTGSPQGARALESWSHARGARYLDGAIVCFPAQIGTSDACIICSGASAAFSEAEPVLSLLAPTLDHVAEAVGAAAAQDCAAVAYFAGGLLGALHGALICEAEGLPVAKVCALFSELSPILGGDVAHLGKTLASGDFDHPTASLKTWSAAISRLAGHATDAGIDSRFPRFAADLFEEGVAQGFGQQEVSALIKVLRARNGAAQ

SEQ ID NO: 74 - DNA, 879 bp, Artificial Sequence
atgcgccatctgagcgtgattggcctgggcgcgatgggccaggcgctggcgaccaccctgctgaaggcaggacacccagtaacagtttggaatcgtggggctgcaaaggctgctccactccaagctctaggtgctactttggctcctagtgttggagccgctatcgccgcgagcgatattaccctggtgtgcgtggataactatgcggtgagccagctgctgctggatgaagcgagcgatgcagtagccgggaagttgcttgtacaactttcgacgggaagtcctcaaggtgcacgtgcccttgagagctggagccatgcgcgcggcgcgcgctatctggatggcgcgattgtttgctttccggcgcagattggcaccagcgatgcgtgtattatttgcagcggcgcgagcgcggcgtttagcgaagcggaaccggtgctgtctctcctcgctcccacactagaccacgttgccgaggctgtgggagcggccgcggctcaagactgcgcggcggttgcgtatttcgctggaggcctgctgggcgcgctgcatggcgcgctgatttgcgaagcggaaggcctgccggtggcgaaagtgtgcgcgctgtttagcgaactgagcccgattctgggcggcgatgtggcgcatctgggcaagacattggcgagcggcgatttcgaccacccgactgcgagcctgaagacttggagcgcggcgattagccgcctggcgggccatgcgaccgatgcgggcattgatagccgctttccgcgctttgcggcggatctgtttgaagaaggcgtggcgcagggctttggccagcaggaagtgagcgcgctgattaaagtgctgcgcgcgcgcaacggcgcggcgcagtaa

SEQ ID NO: 75 - protein, 292 aa, Artificial Sequence
MRHLSVIGLGAMGSALATTLLKAGHPVTVWNRGAAKAAPLQALGATLAPSVGAAIAASDITLVCVDNYAVSQLLLDEASDAVAGKLLVQLSTGSPQGARALESWSHARGARYLDGAILDFPAQIGTSDATIICSGASAAFSEAEPVLSLLAPTLDHVAEAVGAAAAQDCAAVAYFAGGLLGALHGALICEAEGLPVAKVCAAFSELSPILGGDVAHLGKTLASGDFDHPGASLKTWSALISRLAGHATDAGIDSRFPRFAADLFEEGVAQGFGQQEVSALIKVLRARNGAAQ

SEQ ID NO: 76 - DNA, 879 bp, Artificial Sequence
atgcgccatctgagcgtgattggcctgggcgcgatgggcagcgcgctggcgaccaccctgctgaaggcaggacacccagtaacagtttggaatcgtggggctgcaaaggctgctccactccaagctctaggtgctactttggctcctagtgttggagccgctatcgccgcgagcgatattaccctggtgtgcgtggataactatgcggtgagccagctgctgctggatgaagcgagcgatgcagtagccgggaagttgcttgtacaactttcgacgggaagtcctcaaggtgcacgtgcccttgagagctggagccatgcgcgcggcgcgcgctatctggatggcgcgattctggattttccggcgcagattggcaccagcgatgcgactattatttgcagcggcgcgagcgcggcgtttagcgaagcggaaccggtgctgtctctcctcgctcccacactagaccacgttgccgaggctgtgggagcggccgcggctcaagactgcgcggcggttgcgtatttcgctggaggcctgctgggcgcgctgcatggcgcgctgatttgcgaagcggaaggcctgccggtggcgaaagtgtgcgcggcttttagcgaactgagcccgattctgggcggcgatgtggcgcatctgggcaagacattggcgagcggcgatttcgaccacccgggggcgagcctgaagacttggagcgcgctgattagccgcctggcgggccatgcgaccgatgcgggcattgatagccgctttccgcgctttgcggcggatctgtttgaagaaggcgtggcgcagggctttggccagcaggaagtgagcgcgctgattaaagtgctgcgcgcgcgcaacggcgcggcgcagtaa

SEQ ID NO: 77 - protein, 292 aa, Artificial Sequence
MRHLSVIGLGAMGQALATTLLKAGHPVTVWNRAAAKAAPLQALGATLAPSVGAAIAASDITLVCVDNYAVSQLLLDEASDAVAGKLLVQLSTGSPQGARALESWSHARGARYLDGAILCFPAQIGTSDACIICSGASAAFSEAEPVLSLLAPTLDHVAEAVGAAAAQDCAAVAYFAGGLLGALHGALICEAEGLPVAKVCASFSEFSPILGGDVAHLGKTLASGDFDHPLASLKTWSALISRLAGHATDAGIDSRFPRFAADLFEEGVAQGFGQQEVSALIKVLRARNGAAQ

SEQ ID NO: 78 - DNA, 879 bp, Artificial Sequence
atgcgccatctgagcgtgattggcctgggcgcgatgggccaggcgctggcgaccaccctgctgaaggcaggacacccagtaacagtttggaatcgtgcggctgcaaaggctgctccactccaagctctaggtgctactttggctcctagtgttggagccgctatcgccgcgagcgatattaccctggtgtgcgtggataactatgcggtgagccagctgctgctggatgaagcgagcgatgcagtagccgggaagttgcttgtacaactttcgacgggaagtcctcaaggtgcacgtgcccttgagagctggagccatgcgcgcggcgcgcgctatctggatggcgcgattctgtgctttccggcgcagattggcaccagcgatgcgtgtattatttgcagcggcgcgagcgcggcgtttagcgaagcggaaccggtgctgtctctcctcgctcccacactagaccacgttgccgaggctgtgggagcggccgcggctcaagactgcgcggcggttgcgtatttcgctggaggcctgctgggcgcgctgcatggcgcgctgatttgcgaagcggaaggcctgccggtggcgaaagtgtgcgcgagctttagcgaatttagcccgattctgggcggcgatgtggcgcatctgggcaagacattggcgagcggcgatttcgaccacccgctggcgagcctgaagacttggagcgcgctgattagccgcctggcgggccatgcgaccgatgcgggcattgatagccgctttccgcgctttgcggcggatctgtttgaagaaggcgtggcgcagggctttggccagcaggaagtgagcgcgctgattaaagtgctgcgcgcgcgcaacggcgcggcgcagtaa

SEQ ID NO: 79 - protein, 292 aa, Artificial Sequence
MRHLSVIGLGAMGQALATTLLKAGHPVTVWNRGAAKAAPLQALGATLAPSVGAAIAASDITLVCVDNYAVSQLLLDEASDAVAGKLLVQLSTGSPQGARALESWSHARGARYLDGAILDFPAQIGTSDALIICSGASAAFSEAEPVLSLLAPTLDHVAEAVGAAAAQDCAAVAYFAGGLLGALHGALICEAEGLPVAKVCAQFSELSPILGGDVAHLGKTLASGDFDHPGASLFTWSAAISRLAGHATDAGIDSRFPRFAADLFEEGVAQGFGQQEVSALIKVLRARNGAAQ

SEQ ID NO: 80 - DNA, 879 bp, Artificial Sequence
atgcgccatctgagcgtgattggcctgggcgcgatgggccaggcgctggcgaccaccctgctgaaggcaggacacccagtaacagtttggaatcgtggggctgcaaaggctgctccactccaagctctaggtgctactttggctcctagtgttggagccgctatcgccgcgagcgatattaccctggtgtgcgtggataactatgcggtgagccagctgctgctggatgaagcgagcgatgcagtagccgggaagttgcttgtacaactttcgacgggaagtcctcaaggtgcacgtgcccttgagagctggagccatgcgcgcggcgcgcgctatctggatggcgcgattctggattttccggcgcagattggcaccagcgatgcgctgattatttgcagcggcgcgagcgcggcgtttagcgaagcggaaccggtgctgtctctcctcgctcccacactagaccacgttgccgaggctgtgggagcggccgcggctcaagactgcgcggcggttgcgtatttcgctggaggcctgctgggcgcgctgcatggcgcgctgatttgcgaagcggaaggcctgccggtggcgaaagtgtgcgcgcagtttagcgaactgagcccgattctgggcggcgatgtggcgcatctgggcaagacattggcgagcggcgatttcgaccacccgggggcgagcctgtttacttggagcgcggcgattagccgcctggcgggccatgcgaccgatgcgggcattgatagccgctttccgcgctttgcggcggatctgtttgaagaaggcgtggcgcagggctttggccagcaggaagtgagcgcgctgattaaagtgctgcgcgcgcgcaacggcgcggcgcagtaa

SEQ ID NO: 81 - protein, 292 aa, Artificial Sequence
MRHLSVIGLGAMGVALATTLLKAGHPVTVWNRAAAKAAPLQALGATLAPSVGAAIAASDITLVCVDNYAVSQLLLDEASDAVAGKLLVQLSTGSPQGARALESWSHARGARYLDGAILCFPAQIGTSDACIICSGASAAFSEAEPVLSLLAPTLDHVAEAVGAAAAQDCAAVAYFAGGLLGALHGALICEAEGLPVAKVCAQFSELSPLLGGDVAHLGKTLASGDFDHPGASLKTWSAAISRLAGHATDAGIDSRFPRFAADLFEEGVAQGFGQQELSALIKVLRARNGAAQ

SEQ ID NO: 82 - DNA, 879 bp, Artificial Sequence
atgcgccatctgagcgtgattggcctgggcgcgatgggcgttgcgctggcgaccaccctgctgaaggcaggacacccagtaacagtttggaatcgtgcggctgcaaaggctgctccactccaagctctaggtgctactttggctcctagtgttggagccgctatcgccgcgagcgatattaccctggtgtgcgtggataactatgcggtgagccagctgctgctggatgaagcgagcgatgcagtagccgggaagttgcttgtacaactttcgacgggaagtcctcaaggtgcacgtgcccttgagagctggagccatgcgcgcggcgcgcgctatctggatggcgcgattctgtgctttccggcgcagattggcaccagcgatgcgtgtattatttgcagcggcgcgagcgcggcgtttagcgaagcggaaccggtgctgtctctcctcgctcccacactagaccacgttgccgaggctgtgggagcggccgcggctcaagactgcgcggcggttgcgtatttcgctggaggcctgctgggcgcgctgcatggcgcgctgatttgcgaagcggaaggcctgccggtggcgaaagtgtgcgcgcagtttagcgaactgagcccgctgctgggcggcgatgtggcgcatctgggcaagacattggcgagcggcgatttcgaccacccgggggcgagcctgaagacttggagcgcggcgattagccgcctggcgggccatgcgaccgatgcgggcattgatagccgctttccgcgctttgcggcggatctgtttgaagaaggcgtggcgcagggctttggccagcaggaactgagcgcgctgattaaagtgctgcgcgcgcgcaacggcgcggcgcagtaa

SEQ ID NO: 83 - protein, 292 aa, Artificial Sequence
MRHLSVIGLGAMGSALATTLLKAGHPVTVWNRGAAKAAPLQALGATLAPSVGAAIAASDITLVCVDNYAVSQLLLDEASDAVAGKLLVQLSTGSPQGARALESWSHARGARYLDGAIVCFPAQIGTSDALIICSGASAAFSEAEPVLSLLAPTLDHVAEAVGAAAAQDCAAVAYFAGGLLGALHGALICEAEGLPVAKVCAAFSELSPILGGDVAHLGKTLASGDFDHPGASLKTWSAAISRLAGHATDAGIDSRFPRFAADLFEEGVAQGFGQQEVSALIKVLRARNGAAQ

SEQ ID NO: 84 - DNA, 879 bp, Artificial Sequence
atgcgccatctgagcgtgattggcctgggcgcgatgggcagcgcgctggcgaccaccctgctgaaggcaggacacccagtaacagtttggaatcgtggcgctgcaaaggctgctccactccaagctctaggtgctactttggctcctagtgttggagccgctatcgccgcgagcgatattaccctggtgtgcgtggataactatgcggtgagccagctgctgctggatgaagcgagcgatgcagtagccgggaagttgcttgtacaactttcgacgggaagtcctcaaggtgcacgtgcccttgagagctggagccatgcgcgcggcgcgcgctatctggatggcgcgattgtttgctttccggcgcagattggcaccagcgatgcgctgattatttgcagcggcgcgagcgcggcgtttagcgaagcggaaccggtgctgtctctcctcgctcccacactagaccacgttgccgaggctgtgggagcggccgcggctcaagactgcgcggcggttgcgtatttcgctggaggcctgctgggcgcgctgcatggcgcgctgatttgcgaagcggaaggcctgccggtggcgaaagtgtgcgcggcgtttagcgaactgagcccgattctgggcggcgatgtggcgcatctgggcaagacattggcgagcggcgatttcgaccacccgggggcgagcctgaagacttggagcgcggcgattagccgcctggcgggccatgcgaccgatgcgggcattgatagccgctttccgcgctttgcggcggatctgtttgaagaaggcgtggcgcagggctttggccagcaggaagtgagcgcgctgattaaagtgctgcgcgcgcgcaacggcgcggcgcagtaa

SEQ ID NO: 85 - protein, 292 aa, Artificial Sequence
MRHLSVIGLGAMGSALATTLLKAGHPVTVWNRGAAKAAPLQALGATLAPSVGAAIAASDITLVCVDNYAVSQLLLDEASDAVAGKLLVQLSTGSPQGARALESWSHARGARYLDGAIVCFPAQIGTSDACIICSGASAAFSEAEPVLSLLAPTLDHVAEAVGAAAAQDCAAVAYFAGGLLGALHGALICEAEGLPVAKVCAAFSELSPILGGDVAHLGKTLASGDFDHPGASLKSWSAAISRLAGHATDAGIDSRFPRFAADLFEEGVAQGFGQQEVSALIKVLRARNGAAQ

SEQ ID NO: 86 - DNA, 879 bp, Artificial Sequence
atgcgccatctgagcgtgattggcctgggcgcgatgggcagcgcgctggcgaccaccctgctgaaggcaggacacccagtaacagtttggaatcgtggcgctgcaaaggctgctccactccaagctctaggtgctactttggctcctagtgttggagccgctatcgccgcgagcgatattaccctggtgtgcgtggataactatgcggtgagccagctgctgctggatgaagcgagcgatgcagtagccgggaagttgcttgtacaactttcgacgggaagtcctcaaggtgcacgtgcccttgagagctggagccatgcgcgcggcgcgcgctatctggatggcgcgattgtatgctttccggcgcagattggcaccagcgatgcgtgtattatttgcagcggcgcgagcgcggcgtttagcgaagcggaaccggtgctgtctctcctcgctcccacactagaccacgttgccgaggctgtgggagcggccgcggctcaagactgcgcggcggttgcgtatttcgctggaggcctgctgggcgcgctgcatggcgcgctgatttgcgaagcggaaggcctgccggtggcgaaagtgtgcgcggcgtttagcgaactgagcccgattctgggcggcgatgtggcgcatctgggcaagacattggcgagcggcgatttcgaccacccgggggcgagcctgaagagctggagcgcggcgattagccgcctggcgggccatgcgaccgatgcgggcattgatagccgctttccgcgctttgcggcggatctgtttgaagaaggcgtggcgcagggctttggccagcaggaagtgagcgcgctgattaaagtgctgcgcgcgcgcaacggcgcggcgcagtaa

SEQ ID NO: 87 - protein, 292 aa, Artificial Sequence
MRHLSVIGLGAMGQALATTLLKAGHPVTVWNRDAAKAAPLQALGATLAPSVGAAIAASDITLVCVDNYAVSQLLLDEASDAVAGKLLVQLSTGSPQGARALESWSHARGARYLDGAIVCFPAQIGTSDALIICSGASAAFSEAEPVLSLLAPTLDHVAEAVGAAAAQDCAAVAYFAGGLLGALHGALICEAEGLPVAKVCAQFSELSPILGGDVAHLGKTLASGDFDHPGASLLTWSAAISRLAGHATDAGIDSRFPRFAADLFEEGVAQGFGQQEVSALIKVLRARNGAAQ

SEQ ID NO: 88 - DNA, 879 bp, Artificial Sequence
atgcgccatctgagcgtgattggcctgggcgcgatgggccaggcgctggcgaccaccctgctgaaggcaggacacccagtaacagtttggaatcgtgatgctgcaaaggctgctccactccaagctctaggtgctactttggctcctagtgttggagccgctatcgccgcgagcgatattaccctggtgtgcgtggataactatgcggtgagccagctgctgctggatgaagcgagcgatgcagtagccgggaagttgcttgtacaactttcgacgggaagtcctcaaggtgcacgtgcccttgagagctggagccatgcgcgcggcgcgcgctatctggatggcgcgattgtttgctttccggcgcagattggcaccagcgatgcgctgattatttgcagcggcgcgagcgcggcgtttagcgaagcggaaccggtgctgtctctcctcgctcccacactagaccacgttgccgaggctgtgggagcggccgcggctcaagactgcgcggcggttgcgtatttcgctggaggcctgctgggcgcgctgcatggcgcgctgatttgcgaagcggaaggcctgccggtggcgaaagtgtgcgcgcagtttagcgaactgagcccgattctgggcggcgatgtggcgcatctgggcaagacattggcgagcggcgatttcgaccacccgggggcgagcctgctgacttggagcgcggcgattagccgcctggcgggccatgcgaccgatgcgggcattgatagccgctttccgcgctttgcggcggatctgtttgaagaaggcgtggcgcagggctttggccagcaggaagtgagcgcgctgattaaagtgctgcgcgcgcgcaacggcgcggcgcagtaa

SEQ ID NO: 89 - protein, 292 aa, Artificial Sequence
MRHLSVIGLGAMGVALATTLLKAGHPVTVWNRGAAKAAPLQALGATLAPSVGAAIAASDITLVCVDNYAVSQLLLDEASDAVAGKLLVQLSTGSPQGARALESWSHARGARYLDGAILDFPAQIGTSDALIICSGASAAFSEAEPVLSLLAPTLDHVAEAVGAAAAQDCAAVAYFAGGLLGALHGALICEAEGLPVAKVCAQFSELSPILGGDVAHLGKTLASGDFDHPGASLKLWSALISRLAGHATDAGIDSRFPRFAADLFEEGVAQGFGQQEVSALIKVLRARNGAAQ

SEQ ID NO: 90 - DNA, 879 bp, Artificial Sequence
atgcgccatctgagcgtgattggcctgggcgcgatgggcgttgcgctggcgaccaccctgctgaaggcaggacacccagtaacagtttggaatcgtggcgctgcaaaggctgctccactccaagctctaggtgctactttggctcctagtgttggagccgctatcgccgcgagcgatattaccctggtgtgcgtggataactatgcggtgagccagctgctgctggatgaagcgagcgatgcagtagccgggaagttgcttgtacaactttcgacgggaagtcctcaaggtgcacgtgcccttgagagctggagccatgcgcgcggcgcgcgctatctggatggcgcgattctggattttccggcgcagattggcaccagcgatgcgctgattatttgcagcggcgcgagcgcggcgtttagcgaagcggaaccggtgctgtctctcctcgctcccacactagaccacgttgccgaggctgtgggagcggccgcggctcaagactgcgcggcggttgcgtatttcgctggaggcctgctgggcgcgctgcatggcgcgctgatttgcgaagcggaaggcctgccggtggcgaaagtgtgcgcgcagtttagcgaactgagcccgattctgggcggcgatgtggcgcatctgggcaagacattggcgagcggcgatttcgaccacccgggggcgagcctgaagctgtggagcgcgctgattagccgcctggcgggccatgcgaccgatgcgggcattgatagccgctttccgcgctttgcggcggatctgtttgaagaaggcgtggcgcagggctttggccagcaggaagtgagcgcgctgattaaagtgctgcgcgcgcgcaacggcgcggcgcagtaa

SEQ ID NO: 91 - protein, 292 aa, Artificial Sequence
MRHLSVIGLGAMGVALATTLLKAGHPVTVWNRSAAKAAPLQALGATLAPSVGAAIAASDITLVCVDNYAVSQLLLDEASDAVAGKLLVQLSTGSPQGARALESWSHARGARYLDGAIMTFPAQIGTSDALIICSGASAAFSEAEPVLSLLAPTLDHVAEAVGAAAAQDCAAVAYFAGGLLGALHGALICEAEGLPVAKVCAQFSELSPILGGDVAHLGKTLASGDFDHPGASLKTWSAYISRLAGHATDAGIDSRFPRFAADLFEEGVAQGFGQQEVSALIKVLRARNGAAQ

SEQ ID NO: 92 - DNA, 879 bp, Artificial Sequence
atgcgccatctgagcgtgattggcctgggcgcgatgggcgttgcgctggcgaccaccctgctgaaggcaggacacccagtaacagtttggaatcgtagtgctgcaaaggctgctccactccaagctctaggtgctactttggctcctagtgttggagccgctatcgccgcgagcgatattaccctggtgtgcgtggataactatgcggtgagccagctgctgctggatgaagcgagcgatgcagtagccgggaagttgcttgtacaactttcgacgggaagtcctcaaggtgcacgtgcccttgagagctggagccatgcgcgcggcgcgcgctatctggatggcgcgattatgacctttccggcgcagattggcaccagcgatgcgctgattatttgcagcggcgcgagcgcggcgtttagcgaagcggaaccggtgctgtctctcctcgctcccacactagaccacgttgccgaggctgtgggagcggccgcggctcaagactgcgcggcggttgcgtatttcgctggaggcctgctgggcgcgctgcatggcgcgctgatttgcgaagcggaaggcctgccggtggcgaaagtgtgcgcgcagtttagcgaactgagcccgattctgggcggcgatgtggcgcatctgggcaagacattggcgagcggcgatttcgaccacccgggggcgagcctgaagacttggagcgcgtatattagccgcctggcgggccatgcgaccgatgcgggcattgatagccgctttccgcgctttgcggcggatctgtttgaagaaggcgtggcgcagggctttggccagcaggaagtgagcgcgctgattaaagtgctgcgcgcgcgcaacggcgcggcgcagtaa

SEQ ID NO: 93 - protein, 292 aa, Artificial Sequence
MRHLSVIGLGAMGQALATTLLKAGHPVTVWNRNAAKAAPLQALGATLAPSVGAAIAASDITLVCVDNYAVSQLLLDEASDAVAGKLLVQLSTGSPQGARALESWSHARGARYLDGAIVCFPAQIGTSDALIICSGASAAFSEAEPVLSLLAPTLDHVAEAVGAAAAQDCAAFAYFAGGLLGALHGALICEAEGLPVAKVCAQFSEYSPTLGGDVAHLGKTLASGDFDHPGASLLTWSAAISRLAGHATDAGIDSRFPRFAADLFEEGVAQGFGQQEVSALIKVLRARNGAAQ

SEQ ID NO: 94 - DNA, 879 bp, Artificial Sequence
atgcgccatctgagcgtgattggcctgggcgcgatgggccaggcgctggcgaccaccctgctgaaggcaggacacccagtaacagtttggaatcgtaatgctgcaaaggctgctccactccaagctctaggtgctactttggctcctagtgttggagccgctatcgccgcgagcgatattaccctggtgtgcgtggataactatgcggtgagccagctgctgctggatgaagcgagcgatgcagtagccgggaagttgcttgtacaactttcgacgggaagtcctcaaggtgcacgtgcccttgagagctggagccatgcgcgcggcgcgcgctatctggatggcgcgattgtgtgctttccggcgcagattggcaccagcgatgcgctgattatttgcagcggcgcgagcgcggcgtttagcgaagcggaaccggtgctgtctctcctcgctcccacactagaccacgttgccgaggctgtgggagcggccgcggctcaagactgcgcggcgtttgcgtatttcgctggaggcctgctgggcgcgctgcatggcgcgctgatttgcgaagcggaaggcctgccggtggcgaaagtgtgcgcgcagtttagcgaatatagcccgaccctgggcggcgatgtggcgcatctgggcaagacattggcgagcggcgatttcgaccacccgggggcgagcctgctgacttggagcgcggcgattagccgcctggcgggccatgcgaccgatgcgggcattgatagccgctttccgcgctttgcggcggatctgtttgaagaaggcgtggcgcagggctttggccagcaggaagtgagcgcgctgattaaagtgctgcgcgcgcgcaacggcgcggcgcagtaa

SEQ ID NO: 95 - protein, 292 aa, Artificial Sequence
MRHLSVIGLGAMGQALATTLLKAGHPVTVWNRGAAKAAPLQALGATLAPSVGAAIAASDITLVCVDNYAVSQLLLDEASDAVAGKLLVQLSTGSPQGARALESWSHARGARYLDGAIVCFPAQIGTSDALIICSGASAAFSEAEPVLSLLAPTLDHVAEAVGAAAAQDCAAVAYFAGGLLGALHGALICEAEGLPVAKVCALFSELSPILGGDVAHLGKTLASGDFDHPGASLVTWSAAISRLAGHATDAGIDSRFPRFAADLFEEGVAQGFGQQEVSALIKVLRARNGAAQ

SEQ ID NO: 96 - DNA, 879 bp, Artificial Sequence
atgcgccatctgagcgtgattggcctgggcgcgatgggccaggcgctggcgaccaccctgctgaaggcaggacacccagtaacagtttggaatcgtggggctgcaaaggctgctccactccaagctctaggtgctactttggctcctagtgttggagccgctatcgccgcgagcgatattaccctggtgtgcgtggataactatgcggtgagccagctgctgctggatgaagcgagcgatgcagtagccgggaagttgcttgtacaactttcgacgggaagtcctcaaggtgcacgtgcccttgagagctggagccatgcgcgcggcgcgcgctatctggatggcgcgattgtgtgctttccggcgcagattggcaccagcgatgcgctgattatttgcagcggcgcgagcgcggcgtttagcgaagcggaaccggtgctgtctctcctcgctcccacactagaccacgttgccgaggctgtgggagcggccgcggctcaagactgcgcggcggttgcgtatttcgctggaggcctgctgggcgcgctgcatggcgcgctgatttgcgaagcggaaggcctgccggtggcgaaagtgtgcgcgttgtttagcgaactgagcccgattctgggcggcgatgtggcgcatctgggcaagacattggcgagcggcgatttcgaccacccgggggcgagcctggtgacttggagcgcggcgattagccgcctggcgggccatgcgaccgatgcgggcattgatagccgctttccgcgctttgcggcggatctgtttgaagaaggcgtggcgcagggctttggccagcaggaagtgagcgcgctgattaaagtgctgcgcgcgcgcaacggcgcggcgcagtaa

SEQ ID NO: 97 - protein, 292 aa, Artificial Sequence
MRHLSVIGLGAMGLALATTLLKAGHPVTVWNRGAAKAAPLQALGATLAPSVGAAIAASDITLVCVDNYAVSQLLLDEASDAVAGKLLVQLSTGSPQGARALESWSHARGARYLDGAILDFPAQIGTSDACIICSGASAAFSEAEPVLSLLAPTLDHVAEAVGAAAAQDCAAVAYFAGGLLGALHGALICEAEGLPVAKVCAAFSELSPTLGGDVAHLGKTLASGDFDHPGASLKTWSAAISRLAGHATDAGIDSRFPRFAADLFEEGVAQGFGQQELSALIKVLRARNGAAQ

SEQ ID NO: 98 - DNA, 879 bp, Artificial Sequence
atgcgccatctgagcgtgattggcctgggcgcgatgggcctggcgctggcgaccaccctgctgaaggcaggacacccagtaacagtttggaatcgtggggctgcaaaggctgctccactccaagctctaggtgctactttggctcctagtgttggagccgctatcgccgcgagcgatattaccctggtgtgcgtggataactatgcggtgagccagctgctgctggatgaagcgagcgatgcagtagccgggaagttgcttgtacaactttcgacgggaagtcctcaaggtgcacgtgcccttgagagctggagccatgcgcgcggcgcgcgctatctggatggcgcgattctggattttccggcgcagattggcaccagcgatgcgtgtattatttgcagcggcgcgagcgcggcgtttagcgaagcggaaccggtgctgtctctcctcgctcccacactagaccacgttgccgaggctgtgggagcggccgcggctcaagactgcgcggcggttgcgtatttcgctggaggcctgctgggcgcgctgcatggcgcgctgatttgcgaagcggaaggcctgccggtggcgaaagtgtgcgcggcgtttagcgaactgagcccgacactgggcggcgatgtggcgcatctgggcaagacattggcgagcggcgatttcgaccacccgggggcgagcctgaagacttggagcgcggcgattagccgcctggcgggccatgcgaccgatgcgggcattgatagccgctttccgcgctttgcggcggatctgtttgaagaaggcgtggcgcagggctttggccagcaggaactgagcgcgctgattaaagtgctgcgcgcgcgcaacggcgcggcgcagtaa

SEQ ID NO: 99 - protein, 292 aa, Artificial Sequence
MRHLSVIGLGAMGQALATTLLKAGHPVTVWNRGAAKAAPLQALGATLAPSVGAAIAASDITLVCVDNYAVSQLLLDEASDAVAGKLLVQLSTGSPQGARALESWSHARGARYLDGAILCFPAQIGTSDACIICSGASAAFSEAEPVLSLLAPTLDHVAEAVGAAAAQDCAAVAYFAGGLLGALHGALICEAEGLPVAKVCAQFSEFSPILGGDVAHLGKTLASGDFDHPLASLVTWSALISRLAGHATDAGIDSRFPRFAADLFEEGVAQGFGQQEVSALIKVLRARNGAAQ

SEQ ID NO: 100 - DNA, 879 bp, Artificial Sequence
atgcgccatctgagcgtgattggcctgggcgcgatgggccaggcgctggcgaccaccctgctgaaggcaggacacccagtaacagtttggaatcgtggggctgcaaaggctgctccactccaagctctaggtgctactttggctcctagtgttggagccgctatcgccgcgagcgatattaccctggtgtgcgtggataactatgcggtgagccagctgctgctggatgaagcgagcgatgcagtagccgggaagttgcttgtacaactttcgacgggaagtcctcaaggtgcacgtgcccttgagagctggagccatgcgcgcggcgcgcgctatctggatggcgcgattctgtgctttccggcgcagattggcaccagcgatgcgtgcattatttgcagcggcgcgagcgcggcgtttagcgaagcggaaccggtgctgtctctcctcgctcccacactagaccacgttgccgaggctgtgggagcggccgcggctcaagactgcgcggcggttgcgtatttcgctggaggcctgctgggcgcgctgcatggcgcgctgatttgcgaagcggaaggcctgccggtggcgaaagtgtgcgcgcagtttagcgaatttagcccgattctgggcggcgatgtggcgcatctgggcaagacattggcgagcggcgatttcgaccacccgctggcgagcctggttacttggagcgcgctgattagccgcctggcgggccatgcgaccgatgcgggcattgatagccgctttccgcgctttgcggcggatctgtttgaagaaggcgtggcgcagggctttggccagcaggaagtgagcgcgctgattaaagtgctgcgcgcgcgcaacggcgcggcgcagtaa

SEQ ID NO: 101 - protein, 292 aa, Artificial Sequence
MRHLSVIGLGAMGQALATTLLKAGHPVTVWNRQAAKAAPLQALGATLAPSVGAAIAASDITLVCVDNYAVSQLLLDEASDAVAGKLLVQLSTGSPQGARALESWSHARGARYLDGAILDFPAQIGTSDATIICSGASAAFSEAEPVLSLLAPTLDHVAEAVGAAAAQDCAAVAYFAGGLLGALHGALICEAEGLPVAKVCAYFSEYSPILGGDVAHLGKTLASGDFDHPGASLFTWSALISRLAGHATDAGIDSRFPRFAADLFEEGVAQGFGQQEVSALIKVLRARNGAAQ

SEQ ID NO: 102 - DNA, 879 bp, Artificial Sequence
atgcgccatctgagcgtgattggcctgggcgcgatgggccaggcgctggcgaccaccctgctgaaggcaggacacccagtaacagtttggaatcgtcaggctgcaaaggctgctccactccaagctctaggtgctactttggctcctagtgttggagccgctatcgccgcgagcgatattaccctggtgtgcgtggataactatgcggtgagccagctgctgctggatgaagcgagcgatgcagtagccgggaagttgcttgtacaactttcgacgggaagtcctcaaggtgcacgtgcccttgagagctggagccatgcgcgcggcgcgcgctatctggatggcgcgattctggattttccggcgcagattggcaccagcgatgcgactattatttgcagcggcgcgagcgcggcgtttagcgaagcggaaccggtgctgtctctcctcgctcccacactagaccacgttgccgaggctgtgggagcggccgcggctcaagactgcgcggcggttgcgtatttcgctggaggcctgctgggcgcgctgcatggcgcgctgatttgcgaagcggaaggcctgccggtggcgaaagtgtgcgcgtattttagcgaatatagcccgattctgggcggcgatgtggcgcatctgggcaagacattggcgagcggcgatttcgaccacccgggggcgagcctgtttacttggagcgcgctgattagccgcctggcgggccatgcgaccgatgcgggcattgatagccgctttccgcgctttgcggcggatctgtttgaagaaggcgtggcgcagggctttggccagcaggaagtgagcgcgctgattaaagtgctgcgcgcgcgcaacggcgcggcgcagtaa

SEQ ID NO: 103 - protein, 292 aa, Artificial Sequence
MRHLSVIGLGAMGVALATTLLKAGHPVTVWNRGAAKAAPLQALGATLAPSVGAAIAASDITLVCVDNYAVSQLLLDEASDAVAGKLLVQLSTGSPQGARALESWSHARGARYLDGAIVCFPAQIGTSDATIICSGASAAFSEAEPVLSLLAPTLDHVAEAVGAAAAQDCAAVAYFAGGLLGALHGALICEAEGLPVAKVCAQFSELSPTLGGDVAHLGKTLASGDFDHPGASLVLWSALISRLAGHATDAGIDSRFPRFAADLFEEGVAQGFGQQEVSALIKVLRARNGAAQ

SEQ ID NO: 104 - DNA, 879 bp, Artificial Sequence
atgcgccatctgagcgtgattggcctgggcgcgatgggcgttgcgctggcgaccaccctgctgaaggcaggacacccagtaacagtttggaatcgtggggctgcaaaggctgctccactccaagctctaggtgctactttggctcctagtgttggagccgctatcgccgcgagcgatattaccctggtgtgcgtggataactatgcggtgagccagctgctgctggatgaagcgagcgatgcagtagccgggaagttgcttgtacaactttcgacgggaagtcctcaaggtgcacgtgcccttgagagctggagccatgcgcgcggcgcgcgctatctggatggcgcgattgtttgctttccggcgcagattggcaccagcgatgcgactattatttgcagcggcgcgagcgcggcgtttagcgaagcggaaccggtgctgtctctcctcgctcccacactagaccacgttgccgaggctgtgggagcggccgcggctcaagactgcgcggcggttgcgtatttcgctggaggcctgctgggcgcgctgcatggcgcgctgatttgcgaagcggaaggcctgccggtggcgaaagtgtgcgcgcagtttagcgaactgagcccgactctgggcggcgatgtggcgcatctgggcaagacattggcgagcggcgatttcgaccacccgggggcgagcctggttctttggagcgcgctgattagccgcctggcgggccatgcgaccgatgcgggcattgatagccgctttccgcgctttgcggcggatctgtttgaagaaggcgtggcgcagggctttggccagcaggaagtgagcgcgctgattaaagtgctgcgcgcgcgcaacggcgcggcgcagtaa

SEQ ID NO: 105 - protein, 292 aa, Artificial Sequence
MRHLSVIGLGAMGQALATTLLKAGHPVTVWNRGAAKAAPLQALGATLAPSVGAAIAASDITLVCVDNYAVSQLLLDEASDAVAGKLLVQLSTGSPQGARALESWSHARGARYLDGAIVTFPAQIGTSDACIICSGASAAFSEAEPVLSLLAPTLDHVAEAVGAAAAQDCAAVAYFAGGLLGALHGALICEAEGLPVAKVCAAFSELSPFLGGDVAHLGKTLASGDFDHPGASLKLWSALISRLAGHATDAGIDSRFPRFAADLFEEGVAQGFGQQEVSALIKVLRARNGAAQ

SEQ ID NO: 106 - DNA, 879 bp, Artificial Sequence
atgcgccatctgagcgtgattggcctgggcgcgatgggccaggcgctggcgaccaccctgctgaaggcaggacacccagtaacagtttggaatcgtggggctgcaaaggctgctccactccaagctctaggtgctactttggctcctagtgttggagccgctatcgccgcgagcgatattaccctggtgtgcgtggataactatgcggtgagccagctgctgctggatgaagcgagcgatgcagtagccgggaagttgcttgtacaactttcgacgggaagtcctcaaggtgcacgtgcccttgagagctggagccatgcgcgcggcgcgcgctatctggatggcgcgattgttacttttccggcgcagattggcaccagcgatgcgtgcattatttgcagcggcgcgagcgcggcgtttagcgaagcggaaccggtgctgtctctcctcgctcccacactagaccacgttgccgaggctgtgggagcggccgcggctcaagactgcgcggcggttgcgtatttcgctggaggcctgctgggcgcgctgcatggcgcgctgatttgcgaagcggaaggcctgccggtggcgaaagtgtgcgcggcgtttagcgaactgagcccgtttctgggcggcgatgtggcgcatctgggcaagacattggcgagcggcgatttcgaccacccgggggcgagcctgaagctttggagcgcgctgattagccgcctggcgggccatgcgaccgatgcgggcattgatagccgctttccgcgctttgcggcggatctgtttgaagaaggcgtggcgcagggctttggccagcaggaagtgagcgcgctgattaaagtgctgcgcgcgcgcaacggcgcggcgcagtaa

SEQ ID NO: 107 - protein, 292 aa, Artificial Sequence
MRHLSVIGLGAMGQALATTLLKAGHPVTVWNRGAAKAAPLQALGATLAPSVGAAIAASDITLVCVDNYAVSQLLLDEASDAVAGKLLVQLSTGSPQGARALESWSHARGARYLDGAIVCFPAQIGTSDATIICSGASAAFSEAEPVLSLLAPTLDHVAEAVGAAAAQDCAAVAYFAGGLLGALHGALICEAEGLPVAKVCAAFSEFSPILGGDVAHLGKTLASGDFDHPGASLKLWSAAISRLAGHATDAGIDSRFPRFAADLFEEGVAQGFGQQEVSALIKVLRARNGAAQ

SEQ ID NO: 108 - DNA, 879 bp, Artificial Sequence
atgcgccatctgagcgtgattggcctgggcgcgatgggccaagcgctggcgaccaccctgctgaaggcaggacacccagtaacagtttggaatcgtggcgctgcaaaggctgctccactccaagctctaggtgctactttggctcctagtgttggagccgctatcgccgcgagcgatattaccctggtgtgcgtggataactatgcggtgagccagctgctgctggatgaagcgagcgatgcagtagccgggaagttgcttgtacaactttcgacgggaagtcctcaaggtgcacgtgcccttgagagctggagccatgcgcgcggcgcgcgctatctggatggcgcgattgtgtgctttccggcgcagattggcaccagcgatgcgaccattatttgcagcggcgcgagcgcggcgtttagcgaagcggaaccggtgctgtctctcctcgctcccacactagaccacgttgccgaggctgtgggagcggccgcggctcaagactgcgcggcggtggcgtatttcgctggaggcctgctgggcgcgctgcatggcgcgctgatttgcgaagcggaaggcctgccggtggcgaaagtgtgcgcggcgtttagcgaatttagcccgattctgggcggcgatgtggcgcatctgggcaagacattggcgagcggcgatttcgaccacccgggcgcgagcctgaagctgtggagcgcggcgattagccgcctggcgggccatgcgaccgatgcgggcattgatagccgctttccgcgctttgcggcggatctgtttgaagaaggcgtggcgcagggctttggccagcaggaagtgagcgcgctgattaaagtgctgcgcgcgcgcaacggcgcggcgcagtaa

SEQ ID NO: 109 - protein, 292 aa, Artificial Sequence
MRHLSVIGLGAMGSALATTLLKAGHPVTVWNRSAAKAAPLQALGATLAPSVGAAIAASDITLVCVDNYAVSQLLLDEASDAVAGKLLVQLSTGSPQGARALESWSHARGARYLDGAILCFPAQIGTSDASIICSGASAAFSEAEPVLSLLAPTLDHVAEAVGAAAAQDCAANAYFAGGLLGALHGALICEAEGLPVAKVCARFSELSPILGGDVAHLGKTLASGDFDHPYASLKTWSAAISRLAGHATDAGIDSRFPRFAADLFEEGVAQGFGQQEVSALIKVLRARNGAAQ

SEQ ID NO: 110 - DNA, 879 bp, Artificial Sequence
atgcgccatctgagcgtgattggcctgggcgcgatgggcagcgcgctggcgaccaccctgctgaaggcaggacacccagtaacagtttggaatcgtagtgctgcaaaggctgctccactccaagctctaggtgctactttggctcctagtgttggagccgctatcgccgcgagcgatattaccctggtgtgcgtggataactatgcggtgagccagctgctgctggatgaagcgagcgatgcagtagccgggaagttgcttgtacaactttcgacgggaagtcctcaaggtgcacgtgcccttgagagctggagccatgcgcgcggcgcgcgctatctggatggcgcgattctgtgctttccggcgcagattggcaccagcgatgcgagcattatttgcagcggcgcgagcgcggcgtttagcgaagcggaaccggtgctgtctctcctcgctcccacactagaccacgttgccgaggctgtgggagcggccgcggctcaagactgcgcggcgaatgcgtatttcgctggaggcctgctgggcgcgctgcatggcgcgctgatttgcgaagcggaaggcctgccggtggcgaaagtgtgcgcgcgctttagcgaactgagcccgattctgggcggcgatgtggcgcatctgggcaagacattggcgagcggcgatttcgaccacccgtatgcgagcctgaagacttggagcgcggcgattagccgcctggcgggccatgcgaccgatgcgggcattgatagccgctttccgcgctttgcggcggatctgtttgaagaaggcgtggcgcagggctttggccagcaggaagtgagcgcgctgattaaagtgctgcgcgcgcgcaacggcgcggcgcagtaa

SEQ ID NO: 111 - protein, 292 aa, Artificial Sequence
MRHLSVIGLGAMGSALATTLLKAGHPVTVWNRSAAKAAPLQALGATLAPSVGAAIAASDITLVCVDNYAVSQLLLDEASDAVAGKLLVQLSTGSPQGARALESWSHARGARYLDGAILCFPAQIGTSDASIICSGASAAFSEAEPVLSLLAPTLDHVAEAVGAAAAQDCAAFAYFAGGLLGALHGALICEAEGLPVAKVCALFSELSPILGGDVAHLGKTLASGDFDHPGASLKTWSAAISRLAGHATDAGIDSRFPRFAADLFEEGVAQGFGQQEVSALIKVLRARNGAAQ

SEQ ID NO: 112 - DNA, 879 bp, Artificial Sequence
atgcgccatctgagcgtgattggcctgggcgcgatgggcagcgcgctggcgaccaccctgctgaaggcaggacacccagtaacagtttggaatcgtagtgctgcaaaggctgctccactccaagctctaggtgctactttggctcctagtgttggagccgctatcgccgcgagcgatattaccctggtgtgcgtggataactatgcggtgagccagctgctgctggatgaagcgagcgatgcagtagccgggaagttgcttgtacaactttcgacgggaagtcctcaaggtgcacgtgcccttgagagctggagccatgcgcgcggcgcgcgctatctggatggcgcgattctgtgctttccggcgcagattggcaccagcgatgcgagcattatttgcagcggcgcgagcgcggcgtttagcgaagcggaaccggtgctgtctctcctcgctcccacactagaccacgttgccgaggctgtgggagcggccgcggctcaagactgcgcggcgtttgcgtatttcgctggaggcctgctgggcgcgctgcatggcgcgctgatttgcgaagcggaaggcctgccggtggcgaaagtgtgcgcgctgtttagcgaactgagcccgattctgggcggcgatgtggcgcatctgggcaagacattggcgagcggcgatttcgaccacccgggcgcgagcctgaagacttggagcgcggcgattagccgcctggcgggccatgcgaccgatgcgggcattgatagccgctttccgcgctttgcggcggatctgtttgaagaaggcgtggcgcagggctttggccagcaggaagtgagcgcgctgattaaagtgctgcgcgcgcgcaacggcgcggcgcagtaa

SEQ ID NO: 113 - protein, 292 aa, Artificial Sequence
MRHLSVIGLGAMGSALATTLLKAGHPVTVWNRSAAKAAPLQALGATLAPSVGAAIAASDITLVCVDNYAVSQLLLDEASDAVAGKLLVQLSTGSPQGARALESWSHARGARYLDGAILCFPAQIGTSDASIICSGASAAFSEAEPVLSLLAPTLDHVAEAVGAAAAQDCAAVAYFAGGLLGALHGALICEAEGLPVAKVCALFSELSPILGGDVAHLGKTLASGDFDHPGASLKTWSAAISRLAGHATDAGIDSRFPRFAADLFEEGVAQGFGQQEVSALIKVLRARNGAAQ

SEQ ID NO: 114 - DNA, 879 bp, Artificial Sequence
atgcgccatctgagcgtgattggcctgggcgcgatgggcagcgcgctggcgaccaccctgctgaaggcaggacacccagtaacagtttggaatcgtagtgctgcaaaggctgctccactccaagctctaggtgctactttggctcctagtgttggagccgctatcgccgcgagcgatattaccctggtgtgcgtggataactatgcggtgagccagctgctgctggatgaagcgagcgatgcagtagccgggaagttgcttgtacaactttcgacgggaagtcctcaaggtgcacgtgcccttgagagctggagccatgcgcgcggcgcgcgctatctggatggcgcgattctgtgctttccggcgcagattggcaccagcgatgcgagcattatttgcagcggcgcgagcgcggcgtttagcgaagcggaaccggtgctgtctctcctcgctcccacactagaccacgttgccgaggctgtgggagcggccgcggctcaagactgcgcggcggtggcgtatttcgctggaggcctgctgggcgcgctgcatggcgcgctgatttgcgaagcggaaggcctgccggtggcgaaagtgtgcgcgctgtttagcgaactgagcccgattctgggcggcgatgtggcgcatctgggcaagacattggcgagcggcgatttcgaccacccgggcgcgagcctgaagacttggagcgcggcgattagccgcctggcgggccatgcgaccgatgcgggcattgatagccgctttccgcgctttgcggcggatctgtttgaagaaggcgtggcgcagggctttggccagcaggaagtgagcgcgctgattaaagtgctgcgcgcgcgcaacggcgcggcgcagtaa

SEQ ID NO: 115 - protein, 292 aa, Artificial Sequence
MRHLSVIGLGAMGQALATTLLKAGHPVTVWNRAAAKAAPLQALGATLAPSVGAAIAASDITLVCVDNYAVSQLLLDEASDAVAGKLLVQLSTGSPQGARALESWSHARGARYLDGAILCFPAQIGTSDACIICSGASAAFSEAEPVLSLLAPTLDHVAEAVGAAAAQDCAAVAYFAGGLLGALHGALICEAEGLPVAKVCALFSEFSPILGGDVAHLGKTLASGDFDHPGASLKTWSALISRLAGHATDAGIDSRFPRFAADLFEEGVAQGFGQQEVSALIKVLRARNGAAQ

SEQ ID NO: 116 - DNA, 879 bp, Artificial Sequence
atgcgccatctgagcgtgattggcctgggcgcgatgggccaagcgctggcgaccaccctgctgaaggcaggacacccagtaacagtttggaatcgtgcggctgcaaaggctgctccactccaagctctaggtgctactttggctcctagtgttggagccgctatcgccgcgagcgatattaccctggtgtgcgtggataactatgcggtgagccagctgctgctggatgaagcgagcgatgcagtagccgggaagttgcttgtacaactttcgacgggaagtcctcaaggtgcacgtgcccttgagagctggagccatgcgcgcggcgcgcgctatctggatggcgcgattctgtgctttccggcgcagattggcaccagcgatgcgtgcattatttgcagcggcgcgagcgcggcgtttagcgaagcggaaccggtgctgtctctcctcgctcccacactagaccacgttgccgaggctgtgggagcggccgcggctcaagactgcgcggcggtggcgtatttcgctggaggcctgctgggcgcgctgcatggcgcgctgatttgcgaagcggaaggcctgccggtggcgaaagtgtgcgcgctgtttagcgaatttagcccgattctgggcggcgatgtggcgcatctgggcaagacattggcgagcggcgatttcgaccacccgggcgcgagcctgaagacttggagcgcgctgattagccgcctggcgggccatgcgaccgatgcgggcattgatagccgctttccgcgctttgcggcggatctgtttgaagaaggcgtggcgcagggctttggccagcaggaagtgagcgcgctgattaaagtgctgcgcgcgcgcaacggcgcggcgcagtaa

SEQ ID NO: 117 - protein, 292 aa, Artificial Sequence
MRHLSVIGLGAMGQALATTLLKAGHPVTVWNRAAAKAAPLQALGATLAPSVGAAIAASDITLVCVDNYAVSQLLLDEASDAVAGKLLVQLSTGSPQGARALESWSHARGARYLDGAIVCFPAQIGTSDATIICSGASAAFSEAEPVLSLLAPTLDHVAEAVGAAAAQDCAAVAYFAGGLLGALHGALICEAEGLPVAKVCALFSELSPILGGDVAHLGKTLASGDFDHPGASLKTWSAAISRLAGHATDAGIDSRFPRFAADLFEEGVAQGFGQQEVSALIKVLRARNGAAQ

SEQ ID NO: 118 - DNA, 879 bp, Artificial Sequence
atgcgccatctgagcgtgattggcctgggcgcgatgggccaagcgctggcgaccaccctgctgaaggcaggacacccagtaacagtttggaatcgtgcggctgcaaaggctgctccactccaagctctaggtgctactttggctcctagtgttggagccgctatcgccgcgagcgatattaccctggtgtgcgtggataactatgcggtgagccagctgctgctggatgaagcgagcgatgcagtagccgggaagttgcttgtacaactttcgacgggaagtcctcaaggtgcacgtgcccttgagagctggagccatgcgcgcggcgcgcgctatctggatggcgcgattgtgtgctttccggcgcagattggcaccagcgatgcgaccattatttgcagcggcgcgagcgcggcgtttagcgaagcggaaccggtgctgtctctcctcgctcccacactagaccacgttgccgaggctgtgggagcggccgcggctcaagactgcgcggcggtggcgtatttcgctggaggcctgctgggcgcgctgcatggcgcgctgatttgcgaagcggaaggcctgccggtggcgaaagtgtgcgcgctgtttagcgaactgagcccgattctgggcggcgatgtggcgcatctgggcaagacattggcgagcggcgatttcgaccacccgggcgcgagcctgaagacttggagcgcggcgattagccgcctggcgggccatgcgaccgatgcgggcattgatagccgctttccgcgctttgcggcggatctgtttgaagaaggcgtggcgcagggctttggccagcaggaagtgagcgcgctgattaaagtgctgcgcgcgcgcaacggcgcggcgcagtaa

SEQ ID NO: 119 - protein, 292 aa, Artificial Sequence
MRHLSVIGLGAMGVALATTLLKAGHPVTVWNRGAAKAAPLQALGATLAPSVGAAIAASDITLVCVDNYAVSQLLLDEASDAVAGKLLVQLSTGSPQGARALESWSHARGARYLDGAILCFPAQIGTSDATIICSGASAAFSEAEPVLSLLAPTLDHVAEAVGAAAAQDCAAVAYFAGGLLGALHGALICEAEGLPVAKVCALFSELSPTLGGDVAHLGKTLASGDFDHPGASLKTWSAAISRLAGHATDAGIDSRFPRFAADLFEEGVAQGFGQQEVSALIKVLRARNGAAQ

SEQ ID NO: 120 - DNA, 879 bp, Artificial Sequence
atgcgccatctgagcgtgattggcctgggcgcgatgggcgtggcgctggcgaccaccctgctgaaggcaggacacccagtaacagtttggaatcgtggcgctgcaaaggctgctccactccaagctctaggtgctactttggctcctagtgttggagccgctatcgccgcgagcgatattaccctggtgtgcgtggataactatgcggtgagccagctgctgctggatgaagcgagcgatgcagtagccgggaagttgcttgtacaactttcgacgggaagtcctcaaggtgcacgtgcccttgagagctggagccatgcgcgcggcgcgcgctatctggatggcgcgattctgtgctttccggcgcagattggcaccagcgatgcgaccattatttgcagcggcgcgagcgcggcgtttagcgaagcggaaccggtgctgtctctcctcgctcccacactagaccacgttgccgaggctgtgggagcggccgcggctcaagactgcgcggcggtggcgtatttcgctggaggcctgctgggcgcgctgcatggcgcgctgatttgcgaagcggaaggcctgccggtggcgaaagtgtgcgcgctgtttagcgaactgagcccgaccctgggcggcgatgtggcgcatctgggcaagacattggcgagcggcgatttcgaccacccgggcgcgagcctgaagacttggagcgcggcgattagccgcctggcgggccatgcgaccgatgcgggcattgatagccgctttccgcgctttgcggcggatctgtttgaagaaggcgtggcgcagggctttggccagcaggaagtgagcgcgctgattaaagtgctgcgcgcgcgcaacggcgcggcgcagtaa

SEQ ID NO: 121 - protein, 292 aa, Artificial Sequence
MRHLSVIGLGAMGSALATTLLKAGHPVTVWNRGAAKAAPLQALGATLAPSVGAAIAASDITLVCVDNYAVSQLLLDEASDAVAGKLLVQLSTGSPQGARALESWSHARGARYLDGAIVCFPAQIGTSDATIICSGASAAFSEAEPVLSLLAPTLDHVAEAVGAAAAQDCAAVAYFAGGLLGALHGALICEAEGLPVAKVCALFSELSPILGGDVAHLGKTLASGDFDHPGASLLTWSAAISRLAGHATDAGIDSRFPRFAADLFEEGVAQGFGQQEVSALIKVLRARNGAAQ

SEQ ID NO: 122 - DNA, 879 bp, Artificial Sequence
atgcgccatctgagcgtgattggcctgggcgcgatgggcagcgcgctggcgaccaccctgctgaaggcaggacacccagtaacagtttggaatcgtggcgctgcaaaggctgctccactccaagctctaggtgctactttggctcctagtgttggagccgctatcgccgcgagcgatattaccctggtgtgcgtggataactatgcggtgagccagctgctgctggatgaagcgagcgatgcagtagccgggaagttgcttgtacaactttcgacgggaagtcctcaaggtgcacgtgcccttgagagctggagccatgcgcgcggcgcgcgctatctggatggcgcgattgtgtgctttccggcgcagattggcaccagcgatgcgaccattatttgcagcggcgcgagcgcggcgtttagcgaagcggaaccggtgctgtctctcctcgctcccacactagaccacgttgccgaggctgtgggagcggccgcggctcaagactgcgcggcggtggcgtatttcgctggaggcctgctgggcgcgctgcatggcgcgctgatttgcgaagcggaaggcctgccggtggcgaaagtgtgcgcgctgtttagcgaactgagcccgattctgggcggcgatgtggcgcatctgggcaagacattggcgagcggcgatttcgaccacccgggcgcgagcctgctgacttggagcgcggcgattagccgcctggcgggccatgcgaccgatgcgggcattgatagccgctttccgcgctttgcggcggatctgtttgaagaaggcgtggcgcagggctttggccagcaggaagtgagcgcgctgattaaagtgctgcgcgcgcgcaacggcgcggcgcagtaa

SEQ ID NO: 123 - protein, 292 aa, Artificial Sequence
MRHLSVIGLGAMGQALATTLLKAGHPVTVWNRDAAKAAPLQALGATLAPSVGAAIAASDITLVCVDNYAVSQLLLDEASDAVAGKLLVQLSTGSPQGARALESWSHARGARYLDGAILCFPAQIGTSDATIICSGASAAFSEAEPVLSLLAPTLDHVAEAVGAAAAQDCAAVAYFAGGLLGALHGALICEAEGLPVAKVCARFSELSPILGGDVAHLGKTLASGDFDHPGASLLTWSAAISRLAGHATDAGIDSRFPRFAADLFEEGVAQGFGQQEVSALIKVLRARNGAAQ

SEQ ID NO: 124 - DNA, 879 bp, Artificial Sequence
atgcgccatctgagcgtgattggcctgggcgcgatgggccaagcgctggcgaccaccctgctgaaggcaggacacccagtaacagtttggaatcgtgatgctgcaaaggctgctccactccaagctctaggtgctactttggctcctagtgttggagccgctatcgccgcgagcgatattaccctggtgtgcgtggataactatgcggtgagccagctgctgctggatgaagcgagcgatgcagtagccgggaagttgcttgtacaactttcgacgggaagtcctcaaggtgcacgtgcccttgagagctggagccatgcgcgcggcgcgcgctatctggatggcgcgattctgtgctttccggcgcagattggcaccagcgatgcgaccattatttgcagcggcgcgagcgcggcgtttagcgaagcggaaccggtgctgtctctcctcgctcccacactagaccacgttgccgaggctgtgggagcggccgcggctcaagactgcgcggcggtggcgtatttcgctggaggcctgctgggcgcgctgcatggcgcgctgatttgcgaagcggaaggcctgccggtggcgaaagtgtgcgcgcgctttagcgaactgagcccgattctgggcggcgatgtggcgcatctgggcaagacattggcgagcggcgatttcgaccacccgggcgcgagcctgctgacttggagcgcggcgattagccgcctggcgggccatgcgaccgatgcgggcattgatagccgctttccgcgctttgcggcggatctgtttgaagaaggcgtggcgcagggctttggccagcaggaagtgagcgcgctgattaaagtgctgcgcgcgcgcaacggcgcggcgcagtaa

SEQ ID NO: 125 - protein, 292 aa, Artificial Sequence
MRHLSVIGLGAMGVALATTLLKAGHPVTVWNRGAAKAAPLQALGATLAPSVGAAIAASDITLVCVDNYAVSQLLLDEASDAVAGKLLVQLSTGSPQGARALESWSHARGARYLDGAILTFPAQIGTSDATIICSGASAAFSEAEPVLSLLAPTLDHVAEAVGAAAAQDCAANAYFAGGLLGALHGALICEAEGLPVAKVCARFSELSPILGGDVAHLGKTLASGDFDHPGASLKLWSAAISRLAGHATDAGIDSRFPRFAADLFEEGVAQGFGQQEVSALIKVLRARNGAAQ

SEQ ID NO: 126 - DNA, 879 bp, Artificial Sequence
atgcgccatctgagcgtgattggcctgggcgcgatgggcgtggcgctggcgaccaccctgctgaaggcaggacacccagtaacagtttggaatcgtggcgctgcaaaggctgctccactccaagctctaggtgctactttggctcctagtgttggagccgctatcgccgcgagcgatattaccctggtgtgcgtggataactatgcggtgagccagctgctgctggatgaagcgagcgatgcagtagccgggaagttgcttgtacaactttcgacgggaagtcctcaaggtgcacgtgcccttgagagctggagccatgcgcgcggcgcgcgctatctggatggcgcgattctgacctttccggcgcagattggcaccagcgatgcgaccattatttgcagcggcgcgagcgcggcgtttagcgaagcggaaccggtgctgtctctcctcgctcccacactagaccacgttgccgaggctgtgggagcggccgcggctcaagactgcgcggcgaatgcgtatttcgctggaggcctgctgggcgcgctgcatggcgcgctgatttgcgaagcggaaggcctgccggtggcgaaagtgtgcgcgcgctttagcgaactgagcccgattctgggcggcgatgtggcgcatctgggcaagacattggcgagcggcgatttcgaccacccgggcgcgagcctgaagctgtggagcgcggcgattagccgcctggcgggccatgcgaccgatgcgggcattgatagccgctttccgcgctttgcggcggatctgtttgaagaaggcgtggcgcagggctttggccagcaggaagtgagcgcgctgattaaagtgctgcgcgcgcgcaacggcgcggcgcagtaa

SEQ ID NO: 127 - protein, 292 aa, Artificial Sequence
MRHLSVIGLGAMGVALATTLLKAGHPVTVWNRDAAKAAPLQALGATLAPSVGAAIAASDITLVCVDNYAVSQLLLDEASDAVAGKLLVQLSTGSPQGARALESWSHARGARYLDGAILTFPAQIGTSDACIICSGASAAFSEAEPVLSLLAPTLDHVAEAVGAAAAQDCAAFAYFAGGLLGALHGALICEAEGLPVAKVCARFSELSPILGGDVAHLGKTLASGDFDHPGASLKTWSAYISRLAGHATDAGIDSRFPRFAADLFEEGVAQGFGQQEVSALIKVLRARNGAAQ

SEQ ID NO: 128 - DNA, 879 bp, Artificial Sequence
atgcgccatctgagcgtgattggcctgggcgcgatgggcgtggcgctggcgaccaccctgctgaaggcaggacacccagtaacagtttggaatcgtgatgctgcaaaggctgctccactccaagctctaggtgctactttggctcctagtgttggagccgctatcgccgcgagcgatattaccctggtgtgcgtggataactatgcggtgagccagctgctgctggatgaagcgagcgatgcagtagccgggaagttgcttgtacaactttcgacgggaagtcctcaaggtgcacgtgcccttgagagctggagccatgcgcgcggcgcgcgctatctggatggcgcgattctgacctttccggcgcagattggcaccagcgatgcgtgcattatttgcagcggcgcgagcgcggcgtttagcgaagcggaaccggtgctgtctctcctcgctcccacactagaccacgttgccgaggctgtgggagcggccgcggctcaagactgcgcggcgtttgcgtatttcgctggaggcctgctgggcgcgctgcatggcgcgctgatttgcgaagcggaaggcctgccggtggcgaaagtgtgcgcgcgctttagcgaactgagcccgattctgggcggcgatgtggcgcatctgggcaagacattggcgagcggcgatttcgaccacccgggcgcgagcctgaagacttggagcgcgtatattagccgcctggcgggccatgcgaccgatgcgggcattgatagccgctttccgcgctttgcggcggatctgtttgaagaaggcgtggcgcagggctttggccagcaggaagtgagcgcgctgattaaagtgctgcgcgcgcgcaacggcgcggcgcagtaa

SEQ ID NO: 129 - protein, 292 aa, Artificial Sequence
MRHLSVIGLGAMGQALATTLLKAGHPVTVWNRQAAKAAPLQALGATLAPSVGAAIAASDITLVCVDNYAVSQLLLDEASDAVAGKLLVQLSTGSPQGARALESWSHARGARYLDGAIVCFPAQIGTSDATIICSGASAAFSEAEPVLSLLAPTLDHVAEAVGAAAAQDCAANAYFAGGLLGALHGALICEAEGLPVAKVCARFSEYSPTLGGDVAHLGKTLASGDFDHPGASLKTWSAAISRLAGHATDAGIDSRFPRFAADLFEEGVAQGFGQQEVSALIKVLRARNGAAQ

SEQ ID NO: 130 - DNA, 879 bp, Artificial Sequence
atgcgccatctgagcgtgattggcctgggcgcgatgggccaagcgctggcgaccaccctgctgaaggcaggacacccagtaacagtttggaatcgtcaagctgcaaaggctgctccactccaagctctaggtgctactttggctcctagtgttggagccgctatcgccgcgagcgatattaccctggtgtgcgtggataactatgcggtgagccagctgctgctggatgaagcgagcgatgcagtagccgggaagttgcttgtacaactttcgacgggaagtcctcaaggtgcacgtgcccttgagagctggagccatgcgcgcggcgcgcgctatctggatggcgcgattgtgtgctttccggcgcagattggcaccagcgatgcgaccattatttgcagcggcgcgagcgcggcgtttagcgaagcggaaccggtgctgtctctcctcgctcccacactagaccacgttgccgaggctgtgggagcggccgcggctcaagactgcgcggcgaatgcgtatttcgctggaggcctgctgggcgcgctgcatggcgcgctgatttgcgaagcggaaggcctgccggtggcgaaagtgtgcgcgcgctttagcgaatatagcccgaccctgggcggcgatgtggcgcatctgggcaagacattggcgagcggcgatttcgaccacccgggcgcgagcctgaagacttggagcgcggcgattagccgcctggcgggccatgcgaccgatgcgggcattgatagccgctttccgcgctttgcggcggatctgtttgaagaaggcgtggcgcagggctttggccagcaggaagtgagcgcgctgattaaagtgctgcgcgcgcgcaacggcgcggcgcagtaa

SEQ ID NO: 131 - protein, 292 aa, Artificial Sequence; identical to SEQ ID NO: 73

SEQ ID NO: 132 - DNA, 879 bp, Artificial Sequence
atgcgccatctgagcgtgattggcctgggcgcgatgggccaagcgctggcgaccaccctgctgaaggcaggacacccagtaacagtttggaatcgtggcgctgcaaaggctgctccactccaagctctaggtgctactttggctcctagtgttggagccgctatcgccgcgagcgatattaccctggtgtgcgtggataactatgcggtgagccagctgctgctggatgaagcgagcgatgcagtagccgggaagttgcttgtacaactttcgacgggaagtcctcaaggtgcacgtgcccttgagagctggagccatgcgcgcggcgcgcgctatctggatggcgcgattgtgtgctttccggcgcagattggcaccagcgatgcgtgcattatttgcagcggcgcgagcgcggcgtttagcgaagcggaaccggtgctgtctctcctcgctcccacactagaccacgttgccgaggctgtgggagcggccgcggctcaagactgcgcggcggtggcgtatttcgctggaggcctgctgggcgcgctgcatggcgcgctgatttgcgaagcggaaggcctgccggtggcgaaagtgtgcgcgctgtttagcgaactgagcccgattctgggcggcgatgtggcgcatctgggcaagacattggcgagcggcgatttcgaccacccgaccgcgagcctgaagacttggagcgcggcgattagccgcctggcgggccatgcgaccgatgcgggcattgatagccgctttccgcgctttgcggcggatctgtttgaagaaggcgtggcgcagggctttggccagcaggaagtgagcgcgctgattaaagtgctgcgcgcgcgcaacggcgcggcgcagtaa

SEQ ID NO: 133 - protein, 292 aa, Artificial Sequence
MRHLSVIGLGAMGSALATTLLKAGHPVTVWNRSAAKAAPLQALGATLAPSVGAAIAASDITLVCVDNYAVSQLLLDEASDAVAGKLLVQLSTGSPQGARALESWSHARGARYLDGAILCFPAQIGTSDASIICSGASAAFSEAEPVLSLLAPTLDHVAEAVGAAAAQDCAANAYFAGGLLGALHGALICEAEGLPVAKVCARFSELSPILGGEVAHLGKTLASGDFDHPYASLKTWSAAISRLAGHATDAGIDSRFPRFAADLFEEGVAQGFGQQEVSALIKVLRARNGAAQ

SEQ ID NO: 134 - DNA, 879 bp, Artificial Sequence
atgcgccatctgagcgtgattggcctgggcgcgatgggcagcgcgctggcgaccaccctgctgaaggcaggacacccagtaacagtttggaatcgtagtgctgcaaaggctgctccactccaagctctaggtgctactttggctcctagtgttggagccgctatcgccgcgagcgatattaccctggtgtgcgtggataactatgcggtgagccagctgctgctggatgaagcgagcgatgcagtagccgggaagttgcttgtacaactttcgacgggaagtcctcaaggtgcacgtgcccttgagagctggagccatgcgcgcggcgcgcgctatctggatggcgcgattctgtgctttccggcgcagattggcaccagcgatgcgagcattatttgcagcggcgcgagcgcggcgtttagcgaagcggaaccggtgctgtctctcctcgctcccacactagaccacgttgccgaggctgtgggagcggccgcggctcaagactgcgcggcgaatgcgtatttcgctggaggcctgctgggcgcgctgcatggcgcgctgatttgcgaagcggaaggcctgccggtggcgaaagtgtgcgcgcgctttagcgaactgagcccgattctgggcggcgaggtggcgcatctgggcaagacattggcgagcggcgatttcgaccacccgtatgcgagcctgaagacttggagcgcggcgattagccgcctggcgggccatgcgaccgatgcgggcattgatagccgctttccgcgctttgcggcggatctgtttgaagaaggcgtggcgcagggctttggccagcaggaagtgagcgcgctgattaaagtgctgcgcgcgcgcaacggcgcggcgcagtaa

SEQ ID NO: 135 - protein, 292 aa, Artificial Sequence
MRHLSVIGLGAMGSALATTLLKAGHPVTVWNRGAAKAAPLQALGATLAPSVGAAIAASDITLVCVDNYAVSQLLLDEASDAVAGKLLVQLSTGSPQGARALESWSHARGARYLDGAILDFPAQIGTSDATIICSGASAAFSEAEPVLSLLAPTLDHVAEAVGAAAAQDCAAVAYFAGGLLGALHGALICEAEGLPVAKVCAAFSELSPILGGEVAHLGKTLASGDFDHPGASLKTWSALISRLAGHATDAGIDSRFPRFAADLFEEGVAQGFGQQEVSALIKVLRARNGAAQ

SEQ ID NO: 136 - DNA, 879 bp, Artificial Sequence
atgcgccatctgagcgtgattggcctgggcgcgatgggcagcgcgctggcgaccaccctgctgaaggcaggacacccagtaacagtttggaatcgtggcgctgcaaaggctgctccactccaagctctaggtgctactttggctcctagtgttggagccgctatcgccgcgagcgatattaccctggtgtgcgtggataactatgcggtgagccagctgctgctggatgaagcgagcgatgcagtagccgggaagttgcttgtacaactttcgacgggaagtcctcaaggtgcacgtgcccttgagagctggagccatgcgcgcggcgcgcgctatctggatggcgcgattctggattttccggcgcagattggcaccagcgatgcgaccattatttgcagcggcgcgagcgcggcgtttagcgaagcggaaccggtgctgtctctcctcgctcccacactagaccacgttgccgaggctgtgggagcggccgcggctcaagactgcgcggcggtggcgtatttcgctggaggcctgctgggcgcgctgcatggcgcgctgatttgcgaagcggaaggcctgccggtggcgaaagtgtgcgcggcgtttagcgaactgagcccgattctgggcggcgaggtggcgcatctgggcaagacattggcgagcggcgatttcgaccacccgggcgcgagcctgaagacttggagcgcgctgattagccgcctggcgggccatgcgaccgatgcgggcattgatagccgctttccgcgctttgcggcggatctgtttgaagaaggcgtggcgcagggctttggccagcaggaagtgagcgcgctgattaaagtgctgcgcgcgcgcaacggcgcggcgcagtaa

SEQ ID NO: 137 - protein, 292 aa, Artificial Sequence
MRHLSVIGLGAMGQALATTLLKAGHPVTVWNRAAAKAAPLQALGATLAPSVGAAIAASDITLVCVDNYAVSQLLLDEASDAVAGKLLVQLSTGSPQGARALESWSHARGARYLDGAILCFPAQIGTSDACIICSGASAAFSEAEPVLSLLAPTLDHVAEAVGAAAAQDCAAVAYFAGGLLGALHGALICEAEGLPVAKVCASFSEFSPILGGEVAHLGKTLASGDFDHPTASLKTWSALISRLAGHATDAGIDSRFPRFAADLFEEGVAQGFGQQEVSALIKVLRARNGAAQ

SEQ ID NO: 138 - DNA, 879 bp, Artificial Sequence
atgcgccatctgagcgtgattggcctgggcgcgatgggccaagcgctggcgaccaccctgctgaaggcaggacacccagtaacagtttggaatcgtgcggctgcaaaggctgctccactccaagctctaggtgctactttggctcctagtgttggagccgctatcgccgcgagcgatattaccctggtgtgcgtggataactatgcggtgagccagctgctgctggatgaagcgagcgatgcagtagccgggaagttgcttgtacaactttcgacgggaagtcctcaaggtgcacgtgcccttgagagctggagccatgcgcgcggcgcgcgctatctggatggcgcgattctgtgctttccggcgcagattggcaccagcgatgcgtgcattatttgcagcggcgcgagcgcggcgtttagcgaagcggaaccggtgctgtctctcctcgctcccacactagaccacgttgccgaggctgtgggagcggccgcggctcaagactgcgcggcggtggcgtatttcgctggaggcctgctgggcgcgctgcatggcgcgctgatttgcgaagcggaaggcctgccggtggcgaaagtgtgcgcgagctttagcgaatttagcccgattctgggcggcgaggtggcgcatctgggcaagacattggcgagcggcgatttcgaccacccgaccgcgagcctgaagacttggagcgcgctgattagccgcctggcgggccatgcgaccgatgcgggcattgatagccgctttccgcgctttgcggcggatctgtttgaagaaggcgtggcgcagggctttggccagcaggaagtgagcgcgctgattaaagtgctgcgcgcgcgcaacggcgcggcgcagtaa

SEQ ID NO: 139 - protein, 292 aa, Artificial Sequence
MRHLSVIGLGAMGQALATTLLKAGHPVTVWNRGAAKAAPLQALGATLAPSVGAAIAASDITLVCVDNYAVSQLLLDEASDAVAGKLLVQLSTGSPQGARALESWSHARGARYLDGAILDFPAQIGTSDATIICSGASAAFSEAEPVLSLLAPTLDHVAEAVGAAAAQDCAAVAYFAGGLLGALHGALICEAEGLPVAKVCAQFSELSPILGGEVAHLGKTLASGDFDHPGASLFTWSAAISRLAGHATDAGIDSRFPRFAADLFEEGVAQGFGQQEVSALIKVLRARNGAAQ

SEQ ID NO: 140 - DNA, 879 bp, Artificial Sequence
atgcgccatctgagcgtgattggcctgggcgcgatgggccaagcgctggcgaccaccctgctgaaggcaggacacccagtaacagtttggaatcgtggcgctgcaaaggctgctccactccaagctctaggtgctactttggctcctagtgttggagccgctatcgccgcgagcgatattaccctggtgtgcgtggataactatgcggtgagccagctgctgctggatgaagcgagcgatgcagtagccgggaagttgcttgtacaactttcgacgggaagtcctcaaggtgcacgtgcccttgagagctggagccatgcgcgcggcgcgcgctatctggatggcgcgattctggattttccggcgcagattggcaccagcgatgcgaccattatttgcagcggcgcgagcgcggcgtttagcgaagcggaaccggtgctgtctctcctcgctcccacactagaccacgttgccgaggctgtgggagcggccgcggctcaagactgcgcggcggtggcgtatttcgctggaggcctgctgggcgcgctgcatggcgcgctgatttgcgaagcggaaggcctgccggtggcgaaagtgtgcgcgcagtttagcgaactgagcccgattctgggcggcgaggtggcgcatctgggcaagacattggcgagcggcgatttcgaccacccgggcgcgagcctgtttacttggagcgcggcgattagccgcctggcgggccatgcgaccgatgcgggcattgatagccgctttccgcgctttgcggcggatctgtttgaagaaggcgtggcgcagggctttggccagcaggaagtgagcgcgctgattaaagtgctgcgcgcgcgcaacggcgcggcgcagtaa

SEQ ID NO: 141 - protein, 292 aa, Artificial Sequence
MRHLSVIGLGAMGVALATTLLKAGHPVTVWNRAAAKAAPLQALGATLAPSVGAAIAASDITLVCVDNYAVSQLLLDEASDAVAGKLLVQLSTGSPQGARALESWSHARGARYLDGAILCFPAQIGTSDACIICSGASAAFSEAEPVLSLLAPTLDHVAEAVGAAAAQDCAAVAYFAGGLLGALHGALICEAEGLPVAKVCAQFSELSPTLGGEVAHLGKTLASGDFDHPGASLKTWSAAISRLAGHATDAGIDSRFPRFAADLFEEGVAQGFGQQELSALIKVLRARNGAAQ

SEQ ID NO: 142 - DNA, 879 bp, Artificial Sequence
atgcgccatctgagcgtgattggcctgggcgcgatgggcgtggcgctggcgaccaccctgctgaaggcaggacacccagtaacagtttggaatcgtgcggctgcaaaggctgctccactccaagctctaggtgctactttggctcctagtgttggagccgctatcgccgcgagcgatattaccctggtgtgcgtggataactatgcggtgagccagctgctgctggatgaagcgagcgatgcagtagccgggaagttgcttgtacaactttcgacgggaagtcctcaaggtgcacgtgcccttgagagctggagccatgcgcgcggcgcgcgctatctggatggcgcgattctgtgctttccggcgcagattggcaccagcgatgcgtgcattatttgcagcggcgcgagcgcggcgtttagcgaagcggaaccggtgctgtctctcctcgctcccacactagaccacgttgccgaggctgtgggagcggccgcggctcaagactgcgcggcggtggcgtatttcgctggaggcctgctgggcgcgctgcatggcgcgctgatttgcgaagcggaaggcctgccggtggcgaaagtgtgcgcgcagtttagcgaactgagcccgaccctgggcggcgaggtggcgcatctgggcaagacattggcgagcggcgatttcgaccacccgggcgcgagcctgaagacttggagcgcggcgattagccgcctggcgggccatgcgaccgatgcgggcattgatagccgctttccgcgctttgcggcggatctgtttgaagaaggcgtggcgcagggctttggccagcaggaactgagcgcgctgattaaagtgctgcgcgcgcgcaacggcgcggcgcagtaa

SEQ ID NO: 143 - protein, 292 aa, Artificial Sequence
MRHLSVIGLGAMGSALATTLLKAGHPVTVWNRGAAKAAPLQALGATLAPSVGAAIAASDITLVCVDNYAVSQLLLDEASDAVAGKLLVQLSTGSPQGARALESWSHARGARYLDGAIVCFPAQIGTSDATIICSGASAAFSEAEPVLSLLAPTLDHVAEAVGAAAAQDCAAVAYFAGGLLGALHGALICEAEGLPVAKVCAAFSELSPILGGEVAHLGKTLASGDFDHPGASLKTWSAAISRLAGHATDAGIDSRFPRFAADLFEEGVAQGFGQQEVSALIKVLRARNGAAQ

SEQ ID NO: 144 - DNA, 879 bp, Artificial Sequence; identical to SEQ ID NO: 142

SEQ ID NO: 145 - protein, 292 aa, Artificial Sequence
MRHLSVIGLGAMGSALATTLLKAGHPVTVWNRGAAKAAPLQALGATLAPSVGAAIAASDITLVCVDNYAVSQLLLDEASDAVAGKLLVQLSTGSPQGARALESWSHARGARYLDGAIVCFPAQIGTSDACIICSGASAAFSEAEPVLSLLAPTLDHVAEAVGAAAAQDCAAVAYFAGGLLGALHGALICEAEGLPVAKVCARFSELSPILGGEVAHLGKTLASGDFDHPGASLKSWSAAISRLAGHATDAGIDSRFPRFAADLFEEGVAQGFGQQEVSALIKVLRARNGAAQ

SEQ ID NO: 146 - DNA, 879 bp, Artificial Sequence
atgcgccatctgagcgtgattggcctgggcgcgatgggcagcgcgctggcgaccaccctgctgaaggcaggacacccagtaacagtttggaatcgtggcgctgcaaaggctgctccactccaagctctaggtgctactttggctcctagtgttggagccgctatcgccgcgagcgatattaccctggtgtgcgtggataactatgcggtgagccagctgctgctggatgaagcgagcgatgcagtagccgggaagttgcttgtacaactttcgacgggaagtcctcaaggtgcacgtgcccttgagagctggagccatgcgcgcggcgcgcgctatctggatggcgcgattgtgtgctttccggcgcagattggcaccagcgatgcgtgcattatttgcagcggcgcgagcgcggcgtttagcgaagcggaaccggtgctgtctctcctcgctcccacactagaccacgttgccgaggctgtgggagcggccgcggctcaagactgcgcggcggtggcgtatttcgctggaggcctgctgggcgcgctgcatggcgcgctgatttgcgaagcggaaggcctgccggtggcgaaagtgtgcgcgcgctttagcgaactgagcccgattctgggcggcgaggtggcgcatctgggcaagacattggcgagcggcgatttcgaccacccgggcgcgagcctgaagagctggagcgcggcgattagccgcctggcgggccatgcgaccgatgcgggcattgatagccgctttccgcgctttgcggcggatctgtttgaagaaggcgtggcgcagggctttggccagcaggaagtgagcgcgctgattaaagtgctgcgcgcgcgcaacggcgcggcgcagtaa

SEQ ID NO: 147 - protein, 292 aa, Artificial Sequence
MRHLSVIGLGAMGQALATTLLKAGHPVTVWNRDAAKAAPLQALGATLAPSVGAAIAASDITLVCVDNYAVSQLLLDEASDAVAGKLLVQLSTGSPQGARALESWSHARGARYLDGAIVCFPAQIGTSDATIICSGASAAFSEAEPVLSLLAPTLDHVAEAVGAAAAQDCAAVAYFAGGLLGALHGALICEAEGLPVAKVCARFSELSPILGGEVAHLGKTLASGDFDHPGASLLTWSAAISRLAGHATDAGIDSRFPRFAADLFEEGVAQGFGQQEVSALIKVLRARNGAAQ

SEQ ID NO: 148 - DNA, 879 bp, Artificial Sequence
atgcgccatctgagcgtgattggcctgggcgcgatgggccaagcgctggcgaccaccctgctgaaggcaggacacccagtaacagtttggaatcgtgatgctgcaaaggctgctccactccaagctctaggtgctactttggctcctagtgttggagccgctatcgccgcgagcgatattaccctggtgtgcgtggataactatgcggtgagccagctgctgctggatgaagcgagcgatgcagtagccgggaagttgcttgtacaactttcgacgggaagtcctcaaggtgcacgtgcccttgagagctggagccatgcgcgcggcgcgcgctatctggatggcgcgattgtgtgctttccggcgcagattggcaccagcgatgcgaccattatttgcagcggcgcgagcgcggcgtttagcgaagcggaaccggtgctgtctctcctcgctcccacactagaccacgttgccgaggctgtgggagcggccgcggctcaagactgcgcggcggtggcgtatttcgctggaggcctgctgggcgcgctgcatggcgcgctgatttgcgaagcggaaggcctgccggtggcgaaagtgtgcgcgcgctttagcgaactgagcccgattctgggcggcgaggtggcgcatctgggcaagacattggcgagcggcgatttcgaccacccgggcgcgagcctgctgacttggagcgcggcgattagccgcctggcgggccatgcgaccgatgcgggcattgatagccgctttccgcgctttgcggcggatctgtttgaagaaggcgtggcgcagggctttggccagcaggaagtgagcgcgctgattaaagtgctgcgcgcgcgcaacggcgcggcgcagtaa

SEQ ID NO: 149 - protein, 292 aa, Artificial Sequence
MRHLSVIGLGAMGVALATTLLKAGHPVTVWNRGAAKAAPLQALGATLAPSVGAAIAASDITLVCVDNYAVSQLLLDEASDAVAGKLLVQLSTGSPQGARALESWSHARGARYLDGAILDFPAQIGTSDATIICSGASAAFSEAEPVLSLLAPTLDHVAEAVGAAAAQDCAAVAYFAGGLLGALHGALICEAEGLPVAKVCARFSELSPILGGCVAHLGKTLASGDFDHPGASLKLWSALISRLAGHATDAGIDSRFPRFAADLFEEGVAQGFGQQEVSALIKVLRARNGAAQ

SEQ ID NO: 150 - DNA, 879 bp, Artificial Sequence
atgcgccatctgagcgtgattggcctgggcgcgatgggcgtggcgctggcgaccaccctgctgaaggcaggacacccagtaacagtttggaatcgtggcgctgcaaaggctgctccactccaagctctaggtgctactttggctcctagtgttggagccgctatcgccgcgagcgatattaccctggtgtgcgtggataactatgcggtgagccagctgctgctggatgaagcgagcgatgcagtagccgggaagttgcttgtacaactttcgacgggaagtcctcaaggtgcacgtgcccttgagagctggagccatgcgcgcggcgcgcgctatctggatggcgcgattctggattttccggcgcagattggcaccagcgatgcgaccattatttgcagcggcgcgagcgcggcgtttagcgaagcggaaccggtgctgtctctcctcgctcccacactagaccacgttgccgaggctgtgggagcggccgcggctcaagactgcgcggcggtggcgtatttcgctggaggcctgctgggcgcgctgcatggcgcgctgatttgcgaagcggaaggcctgccggtggcgaaagtgtgcgcgcgctttagcgaactgagcccgattctgggcggctgcgtggcgcatctgggcaagacattggcgagcggcgatttcgaccacccgggcgcgagcctgaagctgtggagcgcgctgattagccgcctggcgggccatgcgaccgatgcgggcattgatagccgctttccgcgctttgcggcggatctgtttgaagaaggcgtggcgcagggctttggccagcaggaagtgagcgcgctgattaaagtgctgcgcgcgcgcaacggcgcggcgcagtaa

SEQ ID NO: 151 - protein, 292 aa, Artificial Sequence
MRHLSVIGLGAMGVALATTLLKAGHPVTVWNRRAAKAAPLQALGATLAPSVGAAIAASDITLVCVDNYAVSQLLLDEASDAVAGKLLVQLSTGSPQGARALESWSHARGARYLDGAIMTFPAQIGTSDATIICSGASAAFSEAEPVLSLLAPTLDHVAEAVGAAAAQDCAAFAYFAGGLLGALHGALICEAEGLPVAKVCARFSELSPILGGCVAHLGKTLASGDFDHPGASLKTWSAYISRLAGHATDAGIDSRFPRFAADLFEEGVAQGFGQQEVSALIKVLRARNGAAQ

SEQ ID NO: 152 - DNA, 879 bp, Artificial Sequence
atgcgccatctgagcgtgattggcctgggcgcgatgggcgtggcgctggcgaccaccctgctgaaggcaggacacccagtaacagtttggaatcgtcgcgctgcaaaggctgctccactccaagctctaggtgctactttggctcctagtgttggagccgctatcgccgcgagcgatattaccctggtgtgcgtggataactatgcggtgagccagctgctgctggatgaagcgagcgatgcagtagccgggaagttgcttgtacaactttcgacgggaagtcctcaaggtgcacgtgcccttgagagctggagccatgcgcgcggcgcgcgctatctggatggcgcgattatgacctttccggcgcagattggcaccagcgatgcgaccattatttgcagcggcgcgagcgcggcgtttagcgaagcggaaccggtgctgtctctcctcgctcccacactagaccacgttgccgaggctgtgggagcggccgcggctcaagactgcgcggcgtttgcgtatttcgctggaggcctgctgggcgcgctgcatggcgcgctgatttgcgaagcggaaggcctgccggtggcgaaagtgtgcgcgcgctttagcgaactgagcccgattctgggcggctgcgtggcgcatctgggcaagacattggcgagcggcgatttcgaccacccgggcgcgagcctgaagacttggagcgcgtatattagccgcctggcgggccatgcgaccgatgcgggcattgatagccgctttccgcgctttgcggcggatctgtttgaagaaggcgtggcgcagggctttggccagcaggaagtgagcgcgctgattaaagtgctgcgcgcgcgcaacggcgcggcgcagtaa

SEQ ID NO: 153 - protein, 292 aa, Artificial Sequence
MRHLSVIGLGAMGQALATTLLKAGHPVTVWNRNAAKAAPLQALGATLAPSVGAAIAASDITLVCVDNYAVSQLLLDEASDAVAGKLLVQLSTGSPQGARALESWSHARGARYLDGAIVCFPAQIGTSDATIICSGASAAFSEAEPVLSLLAPTLDHVAEAVGAAAAQDCAAVAYFAGGLLGALHGALICEAEGLPVAKVCAQFSEYSPTLGGCVAHLGKTLASGDFDHPGASLLTWSAAISRLAGHATDAGIDSRFPRFAADLFEEGVAQGFGQQEVSALIKVLRARNGAAQ

SEQ ID NO: 154 - DNA, 879 bp, Artificial Sequence
atgcgccatctgagcgtgattggcctgggcgcgatgggccaagcgctggcgaccaccctgctgaaggcaggacacccagtaacagtttggaatcgtaatgctgcaaaggctgctccactccaagctctaggtgctactttggctcctagtgttggagccgctatcgccgcgagcgatattaccctggtgtgcgtggataactatgcggtgagccagctgctgctggatgaagcgagcgatgcagtagccgggaagttgcttgtacaactttcgacgggaagtcctcaaggtgcacgtgcccttgagagctggagccatgcgcgcggcgcgcgctatctggatggcgcgattgtgtgctttccggcgcagattggcaccagcgatgcgaccattatttgcagcggcgcgagcgcggcgtttagcgaagcggaaccggtgctgtctctcctcgctcccacactagaccacgttgccgaggctgtgggagcggccgcggctcaagactgcgcggcggtggcgtatttcgctggaggcctgctgggcgcgctgcatggcgcgctgatttgcgaagcggaaggcctgccggtggcgaaagtgtgcgcgcagtttagcgaatatagcccgaccctgggcggctgcgtggcgcatctgggcaagacattggcgagcggcgatttcgaccacccgggcgcgagcctgctgacttggagcgcggcgattagccgcctggcgggccatgcgaccgatgcgggcattgatagccgctttccgcgctttgcggcggatctgtttgaagaaggcgtggcgcagggctttggccagcaggaagtgagcgcgctgattaaagtgctgcgcgcgcgcaacggcgcggcgcagtaa

SEQ ID NO: 155 - protein, 292 aa, Artificial Sequence
MRHLSVIGLGAMGQALATTLLKAGHPVTVWNRGAAKAAPLQALGATLAPSVGAAIAASDITLVCVDNYAVSQLLLDEASDAVAGKLLVQLSTGSPQGARALESWSHARGARYLDGAIVCFPAQIGTSDATIICSGASAAFSEAEPVLSLLAPTLDHVAEAVGAAAAQDCAAVAYFAGGLLGALHGALICEAEGLPVAKVCALFSELSPILGGCVAHLGKTLASGDFDHPGASLVTWSAAISRLAGHATDAGIDSRFPRFAADLFEEGVAQGFGQQEVSALIKVLRARNGAAQ

SEQ ID NO: 156 - DNA, 879 bp, Artificial Sequence
atgcgccatctgagcgtgattggcctgggcgcgatgggccaagcgctggcgaccaccctgctgaaggcaggacacccagtaacagtttggaatcgtggcgctgcaaaggctgctccactccaagctctaggtgctactttggctcctagtgttggagccgctatcgccgcgagcgatattaccctggtgtgcgtggataactatgcggtgagccagctgctgctggatgaagcgagcgatgcagtagccgggaagttgcttgtacaactttcgacgggaagtcctcaaggtgcacgtgcccttgagagctggagccatgcgcgcggcgcgcgctatctggatggcgcgattgtgtgctttccggcgcagattggcaccagcgatgcgaccattatttgcagcggcgcgagcgcggcgtttagcgaagcggaaccggtgctgtctctcctcgctcccacactagaccacgttgccgaggctgtgggagcggccgcggctcaagactgcgcggcggtggcgtatttcgctggaggcctgctgggcgcgctgcatggcgcgctgatttgcgaagcggaaggcctgccggtggcgaaagtgtgcgcgctgtttagcgaactgagcccgattctgggcggctgcgtggcgcatctgggcaagacattggcgagcggcgatttcgaccacccgggcgcgagcctggtgacttggagcgcggcgattagccgcctggcgggccatgcgaccgatgcgggcattgatagccgctttccgcgctttgcggcggatctgtttgaagaaggcgtggcgcagggctttggccagcaggaagtgagcgcgctgattaaagtgctgcgcgcgcgcaacggcgcggcgcagtaa

SEQ ID NO: 157 - protein, 292 aa, Artificial Sequence
MRHLSVIGLGAMGLALATTLLKAGHPVTVWNRGAAKAAPLQALGATLAPSVGAAIAASDITLVCVDNYAVSQLLLDEASDAVAGKLLVQLSTGSPQGARALESWSHARGARYLDGAILDFPAQIGTSDACIICSGASAAFSEAEPVLSLLAPTLDHVAEAVGAAAAQDCAAVAYFAGGLLGALHGALICEAEGLPVAKVCAAFSELSPTLGGCVAHLGKTLASGDFDHPGASLKTWSAAISRLAGHATDAGIDSRFPRFAADLFEEGVAQGFGQQELSALIKVLRARNGAAQ

SEQ ID NO: 158 - DNA, 879 bp, Artificial Sequence
atgcgccatctgagcgtgattggcctgggcgcgatgggcctggcgctggcgaccaccctgctgaaggcaggacacccagtaacagtttggaatcgtggcgctgcaaaggctgctccactccaagctctaggtgctactttggctcctagtgttggagccgctatcgccgcgagcgatattaccctggtgtgcgtggataactatgcggtgagccagctgctgctggatgaagcgagcgatgcagtagccgggaagttgcttgtacaactttcgacgggaagtcctcaaggtgcacgtgcccttgagagctggagccatgcgcgcggcgcgcgctatctggatggcgcgattctggattttccggcgcagattggcaccagcgatgcgtgcattatttgcagcggcgcgagcgcggcgtttagcgaagcggaaccggtgctgtctctcctcgctcccacactagaccacgttgccgaggctgtgggagcggccgcggctcaagactgcgcggcggtggcgtatttcgctggaggcctgctgggcgcgctgcatggcgcgctgatttgcgaagcggaaggcctgccggtggcgaaagtgtgcgcggcgtttagcgaactgagcccgaccctgggcggctgcgtggcgcatctgggcaagacattggcgagcggcgatttcgaccacccgggcgcgagcctgaagacttggagcgcggcgattagccgcctggcgggccatgcgaccgatgcgggcattgatagccgctttccgcgctttgcggcggatctgtttgaagaaggcgtggcgcagggctttggccagcaggaactgagcgcgctgattaaagtgctgcgcgcgcgcaacggcgcggcgcagtaa

SEQ ID NO: 159 - protein, 292 aa, Artificial Sequence
MRHLSVIGLGAMGQALATTLLKAGHPVTVWNRGAAKAAPLQALGATLAPSVGAAIAASDITLVCVDNYAVSQLLLDEASDAVAGKLLVQLSTGSPQGARALESWSHARGARYLDGAILCFPAQIGTSDACIICSGASAAFSEAEPVLSLLAPTLDHVAEAVGAAAAQDCAAVAYFAGGLLGALHGALICEAEGLPVAKVCAQFSEFSPILGGHVAHLGKTLASGDFDHPTASLWTWSALISRLAGHATDAGIDSRFPRFAADLFEEGVAQGFGQQEVSALIKVLRARNGAAQ

SEQ ID NO: 160 - DNA, 879 bp, Artificial Sequence
atgcgccatctgagcgtgattggcctgggcgcgatgggccaagcgctggcgaccaccctgctgaaggcaggacacccagtaacagtttggaatcgtggcgctgcaaaggctgctccactccaagctctaggtgctactttggctcctagtgttggagccgctatcgccgcgagcgatattaccctggtgtgcgtggataactatgcggtgagccagctgctgctggatgaagcgagcgatgcagtagccgggaagttgcttgtacaactttcgacgggaagtcctcaaggtgcacgtgcccttgagagctggagccatgcgcgcggcgcgcgctatctggatggcgcgattctgtgctttccggcgcagattggcaccagcgatgcgtgcattatttgcagcggcgcgagcgcggcgtttagcgaagcggaaccggtgctgtctctcctcgctcccacactagaccacgttgccgaggctgtgggagcggccgcggctcaagactgcgcggcggtggcgtatttcgctggaggcctgctgggcgcgctgcatggcgcgctgatttgcgaagcggaaggcctgccggtggcgaaagtgtgcgcgcagtttagcgaatttagcccgattctgggcggccacgtggcgcatctgggcaagacattggcgagcggcgatttcgaccacccgaccgcgagcctgtggacttggagcgcgctgattagccgcctggcgggccatgcgaccgatgcgggcattgatagccgctttccgcgctttgcggcggatctgtttgaagaaggcgtggcgcagggctttggccagcaggaagtgagcgcgctgattaaagtgctgcgcgcgcgcaacggcgcggcgcagtaa

SEQ ID NO: 161 - protein, 292 aa, Artificial Sequence
MRHLSVIGLGAMGQALATTLLKAGHPVTVWNRQAAKAAPLQALGATLAPSVGAAIAASDITLVCVDNYAVSQLLLDEASDAVAGKLLVQLSTGSPQGARALESWSHARGARYLDGAILDFPAQIGTSDATIICSGASAAFSEAEPVLSLLAPTLDHVAEAVGAAAAQDCAAVAYFAGGLLGALHGALICEAEGLPVAKVCAYFSEYSPILGGHVAHLGKTLASGDFDHPGASLFTWSALISRLAGHATDAGIDSRFPRFAADLFEEGVAQGFGQQEVSALIKVLRARNGAAQ

SEQ ID NO: 162 - DNA, 879 bp, Artificial Sequence
atgcgccatctgagcgtgattggcctgggcgcgatgggccaagcgctggcgaccaccctgctgaaggcaggacacccagtaacagtttggaatcgtcaagctgcaaaggctgctccactccaagctctaggtgctactttggctcctagtgttggagccgctatcgccgcgagcgatattaccctggtgtgcgtggataactatgcggtgagccagctgctgctggatgaagcgagcgatgcagtagccgggaagttgcttgtacaactttcgacgggaagtcctcaaggtgcacgtgcccttgagagctggagccatgcgcgcggcgcgcgctatctggatggcgcgattctggattttccggcgcagattggcaccagcgatgcgaccattatttgcagcggcgcgagcgcggcgtttagcgaagcggaaccggtgctgtctctcctcgctcccacactagaccacgttgccgaggctgtgggagcggccgcggctcaagactgcgcggcggtggcgtatttcgctggaggcctgctgggcgcgctgcatggcgcgctgatttgcgaagcggaaggcctgccggtggcgaaagtgtgcgcgtattttagcgaatatagcccgattctgggcggccacgtggcgcatctgggcaagacattggcgagcggcgatttcgaccacccgggcgcgagcctgtttacttggagcgcgctgattagccgcctggcgggccatgcgaccgatgcgggcattgatagccgctttccgcgctttgcggcggatctgtttgaagaaggcgtggcgcagggctttggccagcaggaagtgagcgcgctgattaaagtgctgcgcgcgcgcaacggcgcggcgcagtaa

SEQ ID NO: 163 - protein, 292 aa, Artificial Sequence
MRHLSVIGLGAMGVALATTLLKAGHPVTVWNRGAAKAAPLQALGATLAPSVGAAIAASDITLVCVDNYAVSQLLLDEASDAVAGKLLVQLSTGSPQGARALESWSHARGARYLDGAIVCFPAQIGTSDATIICSGASAAFSEAEPVLSLLAPTLDHVAEAVGAAAAQDCAAVAYFAGGLLGALHGALICEAEGLPVAKVCAQFSELSPTLGGHVAHLGKTLASGDFDHPGASLVLWSALISRLAGHATDAGIDSRFPRFAADLFEEGVAQGFGQQEVSALIKVLRARNGAAQ

SEQ ID NO: 164 - DNA, 879 bp, Artificial Sequence
atgcgccatctgagcgtgattggcctgggcgcgatgggcgtggcgctggcgaccaccctgctgaaggcaggacacccagtaacagtttggaatcgtggcgctgcaaaggctgctccactccaagctctaggtgctactttggctcctagtgttggagccgctatcgccgcgagcgatattaccctggtgtgcgtggataactatgcggtgagccagctgctgctggatgaagcgagcgatgcagtagccgggaagttgcttgtacaactttcgacgggaagtcctcaaggtgcacgtgcccttgagagctggagccatgcgcgcggcgcgcgctatctggatggcgcgattgtgtgctttccggcgcagattggcaccagcgatgcgaccattatttgcagcggcgcgagcgcggcgtttagcgaagcggaaccggtgctgtctctcctcgctcccacactagaccacgttgccgaggctgtgggagcggccgcggctcaagactgcgcggcggtggcgtatttcgctggaggcctgctgggcgcgctgcatggcgcgctgatttgcgaagcggaaggcctgccggtggcgaaagtgtgcgcgcagtttagcgaactgagcccgaccctgggcggccacgtggcgcatctgggcaagacattggcgagcggcgatttcgaccacccgggcgcgagcctggtgctgtggagcgcgctgattagccgcctggcgggccatgcgaccgatgcgggcattgatagccgctttccgcgctttgcggcggatctgtttgaagaaggcgtggcgcagggctttggccagcaggaagtgagcgcgctgattaaagtgctgcgcgcgcgcaacggcgcggcgcagtaa

SEQ ID NO: 165 - protein, 292 aa, Artificial Sequence
MRHLSVIGLGAMGQALATTLLKAGHPVTVWNRGAAKAAPLQALGATLAPSVGAAIAASDITLVCVDNYAVSQLLLDEASDAVAGKLLVQLSTGSPQGARALESWSHARGARYLDGAIVTFPAQIGTSDACIICSGASAAFSEAEPVLSLLAPTLDHVAEAVGAAAAQDCAAVAYFAGGLLGALHGALICEAEGLPVAKVCAAFSELSPFLGGHVAHLGKTLASGDFDHPGASLKLWSALISRLAGHATDAGIDSRFPRFAADLFEEGVAQGFGQQEVSALIKVLRARNGAAQ

SEQ ID NO: 166 - DNA, 879 bp, Artificial Sequence
atgcgccatctgagcgtgattggcctgggcgcgatgggccaagcgctggcgaccaccctgctgaaggcaggacacccagtaacagtttggaatcgtggcgctgcaaaggctgctccactccaagctctaggtgctactttggctcctagtgttggagccgctatcgccgcgagcgatattaccctggtgtgcgtggataactatgcggtgagccagctgctgctggatgaagcgagcgatgcagtagccgggaagttgcttgtacaactttcgacgggaagtcctcaaggtgcacgtgcccttgagagctggagccatgcgcgcggcgcgcgctatctggatggcgcgattgtgacctttccggcgcagattggcaccagcgatgcgtgcattatttgcagcggcgcgagcgcggcgtttagcgaagcggaaccggtgctgtctctcctcgctcccacactagaccacgttgccgaggctgtgggagcggccgcggctcaagactgcgcggcggtggcgtatttcgctggaggcctgctgggcgcgctgcatggcgcgctgatttgcgaagcggaaggcctgccggtggcgaaagtgtgcgcggcgtttagcgaactgagcccgtttctgggcggccacgtggcgcatctgggcaagacattggcgagcggcgatttcgaccacccgggcgcgagcctgaagctgtggagcgcgctgattagccgcctggcgggccatgcgaccgatgcgggcattgatagccgctttccgcgctttgcggcggatctgtttgaagaaggcgtggcgcagggctttggccagcaggaagtgagcgcgctgattaaagtgctgcgcgcgcgcaacggcgcggcgcagtaa

SEQ ID NO: 167 - protein, 292 aa, Artificial Sequence
MRHLSVIGLGAMGQALATTLLKAGHPVTVWNRGAAKAAPLQALGATLAPSVGAAIAASDITLVCVDNYAVSQLLLDEASDAVAGKLLVQLSTGSPQGARALESWSHARGARYLDGAIVCFPAQIGTSDATIICSGASAAFSEAEPVLSLLAPTLDHVAEAVGAAAAQDCAAVAYFAGGLLGALHGALICEAEGLPVAKVCAAFSEFSPILGGHVAHLGKTLASGDFDHPGASLKLWSAAISRLAGHATDAGIDSRFPRFAADLFEEGVAQGFGQQEVSALIKVLRARNGAAQ

SEQ ID NO: 168 - DNA, 879 bp, Artificial Sequence
atgcgccatctgagcgtgattggcctgggcgcgatgggccaagcgctggcgaccaccctgctgaaggcaggacacccagtaacagtttggaatcgtggcgctgcaaaggctgctccactccaagctctaggtgctactttggctcctagtgttggagccgctatcgccgcgagcgatattaccctggtgtgcgtggataactatgcggtgagccagctgctgctggatgaagcgagcgatgcagtagccgggaagttgcttgtacaactttcgacgggaagtcctcaaggtgcacgtgcccttgagagctggagccatgcgcgcggcgcgcgctatctggatggcgcgattgtgtgctttccggcgcagattggcaccagcgatgcgaccattatttgcagcggcgcgagcgcggcgtttagcgaagcggaaccggtgctgtctctcctcgctcccacactagaccacgttgccgaggctgtgggagcggccgcggctcaagactgcgcggcggtggcgtatttcgctggaggcctgctgggcgcgctgcatggcgcgctgatttgcgaagcggaaggcctgccggtggcgaaagtgtgcgcggcgtttagcgaatttagcccgattctgggcggccacgtggcgcatctgggcaagacattggcgagcggcgatttcgaccacccgggcgcgagcctgaagctgtggagcgcggcgattagccgcctggcgggccatgcgaccgatgcgggcattgatagccgctttccgcgctttgcggcggatctgtttgaagaaggcgtggcgcagggctttggccagcaggaagtgagcgcgctgattaaagtgctgcgcgcgcgcaacggcgcggcgcagtaa

SEQ ID NO: 169 - DNA, 30 bp, Artificial Sequence
tatacatatgcgccatctgagcgtgattgg

SEQ ID NO: 170 - DNA, 29 bp, Artificial Sequence
ttcggatccttactgcgccgcgccgttgc

SEQ ID NO: 171 - DNA, 35 bp, Artificial Sequence
gccggatccaataattttgtttaactttaagaagg

SEQ ID NO: 172 - DNA, 31 bp, Artificial Sequence
ggctcgagttagccacgacccgcttgaaagc

SEQ ID NO: 173 - DNA, 1707 bp, Artificial Sequence
atgcgccatctgagcgtgattggcctgggcgcgatgggcagcgcgctggcgaccaccctgctgaaggcaggacacccagtaacagtttggaatcgtagtgctgcaaaggctgctccactccaagctctaggtgctactttggctcctagtgttggagccgctatcgccgcgagcgatattaccctggtgtgcgtggataactatgcggtgagccagctgctgctggatgaagcgagcgatgcagtagccgggaagttgcttgtacaactttcgacgggaagtcctcaaggtgcacgtgcccttgagagctggagccatgcgcgcggcgcgcgctatctggatggcgcgattctgtgctttccggcgcagattggcaccagcgatgcgagcattatttgcagcggcgcgagcgcggcgtttagcgaagcggaaccggtgctgtctctcctcgctcccacactagaccacgttgccgaggctgtgggagcggccgcggctcaagactgcgcggtggcggcgtatttcgctggaggcctgctgggcgcgctgcatggcgcgctgatttgcgaagcggaaggcctgccggtggcgaaagtgtgcgcgcagtttagcgaactgagcccgattctgggcggcgatgtggcgcatctgggcaagacattggcgagcggcgatttcgaccacccgtatgcgagcctgaagacttggagcgcggcgattagccgcctggcgggccatgcgaccgatgcgggcattgatagccgctttccgcgctttgcggcggatctgtttgaagaaggcgtggcgcagggctttggccagcaggaagtgagcgcgctgattaaagtgctgcgcgcgcgcaacggcgcggcgcagtaaggatccaataattttgtttaactttaagaaggagatatacatatgtacaaggacctggaaggcaaagtggttgtgatcaccggcagcagcaccggtctgggcaagagcatggcgattcgtttcgcgaccgagaaggcgaaagttgtggttaactatcgtagcaaagaggatgaagcgaacagcgtgctggaggaaatcaagaaagttggtggcgaagcgattgcggtgaagggtgacgtgaccgttgagagcgatgtgatcaacctggttcagagcgcgattaaggaatttggtaaactggacgttatgatcaacaacgcgggcctggaaaacccggtgagcagccacgagatgagcctgagcgactggaacaaggttatcgataccaacctgaccggtgcgttcctgggcagccgtgaagcgattaagtactttgtggagaacgatatcaaaggtaccgtgattaacatgagcagcgttcacgagaaaatcccgtggccgctgttcgttcactacgcggcgagcaagggtggcatgaaactgatgaccgagaccctggcgctggaatatgcgccgaagggcatccgtgttaacaacattggtccgggcgcgatcaacaccccgattaacgcggagaaatttgcggacccggaacaacgtgcggatgtggagagcatgatcccgatgggttatattggcgaaccggaagaaattgcggcggttgcggcgtggctggcgagcagcgaggcgagctacgtgaccggtattaccctgttcgcggacggtggcatgacccagtatccgagctttcaagcgggtcgtggctaa